European Patent Application EP 4 112 124 A1, published January 4, 2023. Title: ANTIGEN PRESENTING EXTRACELLUAR VESICLES, COMPOSITIONS COMPRISING THEREOF, AND METHODS FOR MANUFACTURING THEREOF. Applicant: NATIONAL UNIVERSITY CORPORATION KANAZAWA UNIVERSITY NISSAN CHEMICAL CORPORATION. The sequence listing filed with the application follows.

SEQUENCE LISTING (150 sequences)

SEQ ID NO: 1 - protein, 20 aa, Mus musculus
MARSVTLVFLVLVSLTGLYA

SEQ ID NO: 2 - DNA, 60 bp, Mus musculus
atggctcgctcggtgaccctggtctttctggtgcttgtctcactgaccggcctgtatgct

SEQ ID NO: 3 - protein, 8 aa, Artificial Sequence
  peptide sequence derived from OVA
SIINFEKL

SEQ ID NO: 4 - DNA, 24 bp, Artificial Sequence
  DNA sequence derived from OVA
tccattataaattttgaaaagttg

SEQ ID NO: 5 - protein, 15 aa, Artificial Sequence
  synthesized peptide sequence
GGGASGGGGSGGGGS

SEQ ID NO: 6 - DNA, 45 bp, Artificial Sequence
  synthesized DNA sequence
ggcggaggtgcctctggcggtgggggcagcggtggagggggcagt

SEQ ID NO: 7 - protein, 99 aa, Mus musculus [sequence omitted]

SEQ ID NO: 8 - DNA, 297 bp, Mus musculus
atccagaaaacccctcaaattcaagtatactcacgccacccaccggagaatgggaagccgaacatactgaactgctacgtaacacagttccacccgcctcacattgaaatccaaatgctgaagaacgggaaaaaaattcctaaagtagagatgtcagatatgtccttcagcaaggactggtctttctatatcctggctcacactgaattcacccccactgagactgatacatacgcctgcagagttaagcatgccagtatggccgagcccaagaccgtctactgggatcgagacatg

SEQ ID NO: 9 - protein, 348 aa, Mus musculus
GPHSLRYFVTAVSRPGLGEPRYMEVGYVDDTEFVRFDSDAENPRYEPRARWMEQEGPEYWERETQKAKGNEQSFRVDLRTLLGYYNQSKGGSHTIQVISGCEVGSDGRLLRGYQQYAYDGCDYIALNEDLKTWTAADMAALITKHKWEQAGEAERLRAYLEGTCVEWLRRYLKNGNATLLRTDSPKAHVTHHSRPEDKVTLRCWALGFYPADITLTWQLNGEELIQDMELVETRPAGDGTFQKWASVVVPLGKEQYYTCHVYHQGLPEPLTLRWEPPPSTVSNMATVAVLVVLGAAIVTGAVVAFVMKMRRRNTGGKGGDYALAPGSQTSDLSLPDCKVMVHDPHSLA

SEQ ID NO: 10 - DNA, 1044 bp, Mus musculus
ggcccacactcgctgaggtatttcgtcaccgccgtgtcccggcccggcctcggggagccccggtacatggaagtcggctacgtggacgacacggagttcgtgcgcttcgacagcgacgcggagaatccgagatatgagccgcgggcgcggtggatggagcaggaggggcccgagtattgggagcgggagacacagaaagccaagggcaatgagcagagtttccgagtggacctgaggaccctgctcggctactacaaccagagcaagggcggctctcacactattcaggtgatctctggctgtgaagtggggtccgacgggcgactcctccgcgggtaccagcagtacgcctacgacggctgcgattacatcgccctgaacgaagacctgaaaacgtggacggcggcggacatggcggcgctgatcaccaaacacaagtgggagcaggctggtgaagcagagagactcagggcctacctggagggcacgtgcgtggagtggctccgcagatacctgaagaacgggaacgcgacgctgctgcgcacagattccccaaaggcccatgtgacccatcacagcagacctgaagataaagtcaccctgaggtgctgggccctgggcttctaccctgctgacatcaccctgacctggcagttgaatggggaggagctgatccaggacatggagcttgtggagaccaggcctgcaggggatggaaccttccagaagtgggcatctgtggtggtgcctcttgggaaggagcagtattacacatgccatgtgtaccatcaggggctgcctgagcccctcaccctgagatgggagcctcctccatccactgtctccaacatggcgaccgttgctgttctggttgtccttggagctgcaatagtcactggagctgtggtggcttttgtgatgaagatgagaaggagaaacacaggtggaaaaggaggggactatgctctggctccaggctcccagacctctgatctgtctctcccagattgtaaagtgatggttcatgaccctcattctctagcg

SEQ ID NO: 11 - protein, 20 aa, Artificial Sequence
  synthesized peptide sequence
GGGGSGGGGSGGGGSGGGGS

SEQ ID NO: 12 - DNA, 60 bp, Artificial Sequence
  synthesized DNA sequence
ggggggggaggctccggtggaggggggtctggagggggggggtctggtggaggcggaagt

SEQ ID NO: 13 - protein, 510 aa, Artificial Sequence
  peptide sequence derived from OVA, mus musculus
MARSVTLVFLVLVSLTGLYASIINFEKLGGGASGGGGSGGGGSIQKTPQIQVYSRHPPENGKPNILNCYVTQFHPPHIEIQMLKNGKKIPKVEMSDMSFSKDWSFYILAHTEFTPTETDTYACRVKHASMAEPKTVYWDRDMGGGGSGGGGSGGGGSGGGGSGPHSLRYFVTAVSRPGLGEPRYMEVGYVDDTEFVRFDSDAENPRYEPRARWMEQEGPEYWERETQKAKGNEQSFRVDLRTLLGYYNQSKGGSHTIQVISGCEVGSDGRLLRGYQQYAYDGCDYIALNEDLKTWTAADMAALITKHKWEQAGEAERLRAYLEGTCVEWLRRYLKNGNATLLRTDSPKAHVTHHSRPEDKVTLRCWALGFYPADITLTWQLNGEELIQDMELVETRPAGDGTFQKWASVVVPLGKEQYYTCHVYHQGLPEPLTLRWEPPPSTVSNMATVAVLVVLGAAIVTGAVVAFVMKMRRRNTGGKGGDYALAPGSQTSDLSLPDCKVMVHDPHSLA

SEQ ID NO: 14 - DNA, 1530 bp, Artificial Sequence
  DNA sequence derived from OVA, mus musculus
atggctcgctcggtgaccctggtctttctggtgcttgtctcactgaccggcctgtatgcttccattataaattttgaaaagttgggcggaggtgcctctggcggtgggggcagcggtggagggggcagtatccagaaaacccctcaaattcaagtatactcacgccacccaccggagaatgggaagccgaacatactgaactgctacgtaacacagttccacccgcctcacattgaaatccaaatgctgaagaacgggaaaaaaattcctaaagtagagatgtcagatatgtccttcagcaaggactggtctttctatatcctggctcacactgaattcacccccactgagactgatacatacgcctgcagagttaagcatgccagtatggccgagcccaagaccgtctactgggatcgagacatgggggggggaggctccggtggaggggggtctggagggggggggtctggtggaggcggaagtggcccacactcgctgaggtatttcgtcaccgccgtgtcccggcccggcctcggggagccccggtacatggaagtcggctacgtggacgacacggagttcgtgcgcttcgacagcgacgcggagaatccgagatatgagccgcgggcgcggtggatggagcaggaggggcccgagtattgggagcgggagacacagaaagccaagggcaatgagcagagtttccgagtggacctgaggaccctgctcggctactacaaccagagcaagggcggctctcacactattcaggtgatctctggctgtgaagtggggtccgacgggcgactcctccgcgggtaccagcagtacgcctacgacggctgcgattacatcgccctgaacgaagacctgaaaacgtggacggcggcggacatggcggcgctgatcaccaaacacaagtgggagcaggctggtgaagcagagagactcagggcctacctggagggcacgtgcgtggagtggctccgcagatacctgaagaacgggaacgcgacgctgctgcgcacagattccccaaaggcccatgtgacccatcacagcagacctgaagataaagtcaccctgaggtgctgggccctgggcttctaccctgctgacatcaccctgacctggcagttgaatggggaggagctgatccaggacatggagcttgtggagaccaggcctgcaggggatggaaccttccagaagtgggcatctgtggtggtgcctcttgggaaggagcagtattacacatgccatgtgtaccatcaggggctgcctgagcccctcaccctgagatgggagcctcctccatccactgtctccaacatggcgaccgttgctgttctggttgtccttggagctgcaatagtcactggagctgtggtggcttttgtgatgaagatgagaaggagaaacacaggtggaaaaggaggggactatgctctggctccaggctcccagacctctgatctgtctctcccagattgtaaagtgatggttcatgaccctcattctctagcg

SEQ ID NO: 15 - protein, 236 aa, Mus musculus
MGVEGCTKCIKYLLFVFNFVFWLAGGVILGVALWLRHDPQTTSLLYLELGNKPAPNTFYVGIYILIAVGAVMMFVGFLGCYGAIQESQCLLGTFFTCLVILFACEVAAGIWGFVNKDQIAKDVKQFYDQALQQAVMDDDANNAKAVVKTFHETLNCCGSNALTTLTTTILRNSLCPSGGNILTPLLQQDCHQKIDELFSGKLYLIGIAAIVVAVIMIFEMILSMVLCCGIRNSSVY

SEQ ID NO: 16 - DNA, 711 bp, Mus musculus
atgggggtggagggctgcaccaaatgcatcaaatacctgctcttcgtcttcaatttcgtcttctggctggctggaggcgtgatcctaggtgtagctctgtggttgcgtcatgatccacagaccaccagcctgctgtacctggaactgggaaacaaaccggcacccaacaccttctacgtgggcatctacattctcattgctgtgggagctgtgatgatgtttgtaggcttcctggggtgctatggggccatccaggagtcccagtgtctgctggggacgttcttcacctgccttgtgatcctgtttgcctgtgaggtggctgcaggcatctggggcttcgtaaacaaagaccagatcgccaaggatgtgaagcagttctatgaccaggcccttcagcaagctgtgatggatgatgatgccaacaatgccaaggctgtggtgaagactttccatgagacgctcaactgttgtggctccaacgcactgaccacactgactaccaccatactgaggaacagcctgtgtccctcaggcggcaacatactcacccccttactgcagcaagattgtcatcagaaaatcgatgagctcttctctgggaagctgtacctcattggaattgcagccattgtggtagctgtcattatgatctttgagatgattctgagcatggtgctgtgctgtggcatccggaacagctccgtgtactga

SEQ ID NO: 17 - protein, 746 aa, Artificial Sequence
  peptide sequence derived from OVA, mus musculus
MARSVTLVFLVLVSLTGLYASIINFEKLGGGASGGGGSGGGGSIQKTPQIQVYSRHPPENGKPNILNCYVTQFHPPHIEIQMLKNGKKIPKVEMSDMSFSKDWSFYILAHTEFTPTETDTYACRVKHASMAEPKTVYWDRDMGGGGSGGGGSGGGGSGGGGSGPHSLRYFVTAVSRPGLGEPRYMEVGYVDDTEFVRFDSDAENPRYEPRARWMEQEGPEYWERETQKAKGNEQSFRVDLRTLLGYYNQSKGGSHTIQVISGCEVGSDGRLLRGYQQYAYDGCDYIALNEDLKTWTAADMAALITKHKWEQAGEAERLRAYLEGTCVEWLRRYLKNGNATLLRTDSPKAHVTHHSRPEDKVTLRCWALGFYPADITLTWQLNGEELIQDMELVETRPAGDGTFQKWASVVVPLGKEQYYTCHVYHQGLPEPLTLRWEPPPSTVSNMATVAVLVVLGAAIVTGAVVAFVMKMRRRNTGGKGGDYALAPGSQTSDLSLPDCKVMVHDPHSLAMGVEGCTKCIKYLLFVFNFVFWLAGGVILGVALWLRHDPQTTSLLYLELGNKPAPNTFYVGIYILIAVGAVMMFVGFLGCYGAIQESQCLLGTFFTCLVILFACEVAAGIWGFVNKDQIAKDVKQFYDQALQQAVMDDDANNAKAVVKTFHETLNCCGSNALTTLTTTILRNSLCPSGGNILTPLLQQDCHQKIDELFSGKLYLIGIAAIVVAVIMIFEMILSMVLCCGIRNSSVY

SEQ ID NO: 18 - DNA, 2241 bp, Artificial Sequence
  DNA sequence derived from OVA, mus musculus
atggctcgctcggtgaccctggtctttctggtgcttgtctcactgaccggcctgtatgcttccattataaattttgaaaagttgggcggaggtgcctctggcggtgggggcagcggtggagggggcagtatccagaaaacccctcaaattcaagtatactcacgccacccaccggagaatgggaagccgaacatactgaactgctacgtaacacagttccacccgcctcacattgaaatccaaatgctgaagaacgggaaaaaaattcctaaagtagagatgtcagatatgtccttcagcaaggactggtctttctatatcctggctcacactgaattcacccccactgagactgatacatacgcctgcagagttaagcatgccagtatggccgagcccaagaccgtctactgggatcgagacatgggggggggaggctccggtggaggggggtctggagggggggggtctggtggaggcggaagtggcccacactcgctgaggtatttcgtcaccgccgtgtcccggcccggcctcggggagccccggtacatggaagtcggctacgtggacgacacggagttcgtgcgcttcgacagcgacgcggagaatccgagatatgagccgcgggcgcggtggatggagcaggaggggcccgagtattgggagcgggagacacagaaagccaagggcaatgagcagagtttccgagtggacctgaggaccctgctcggctactacaaccagagcaagggcggctctcacactattcaggtgatctctggctgtgaagtggggtccgacgggcgactcctccgcgggtaccagcagtacgcctacgacggctgcgattacatcgccctgaacgaagacctgaaaacgtggacggcggcggacatggcggcgctgatcaccaaacacaagtgggagcaggctggtgaagcagagagactcagggcctacctggagggcacgtgcgtggagtggctccgcagatacctgaagaacgggaacgcgacgctgctgcgcacagattccccaaaggcccatgtgacccatcacagcagacctgaagataaagtcaccctgaggtgctgggccctgggcttctaccctgctgacatcaccctgacctggcagttgaatggggaggagctgatccaggacatggagcttgtggagaccaggcctgcaggggatggaaccttccagaagtgggcatctgtggtggtgcctcttgggaaggagcagtattacacatgccatgtgtaccatcaggggctgcctgagcccctcaccctgagatgggagcctcctccatccactgtctccaacatggcgaccgttgctgttctggttgtccttggagctgcaatagtcactggagctgtggtggcttttgtgatgaagatgagaaggagaaacacaggtggaaaaggaggggactatgctctggctccaggctcccagacctctgatctgtctctcccagattgtaaagtgatggttcatgaccctcattctctagcgatgggggtggagggctgcaccaaatgcatcaaatacctgctcttcgtcttcaatttcgtcttctggctggctggaggcgtgatcctaggtgtagctctgtggttgcgtcatgatccacagaccaccagcctgctgtacctggaactgggaaacaaaccggcacccaacaccttctacgtgggcatctacattctcattgctgtgggagctgtgatgatgtttgtaggcttcctggggtgctatggggccatccaggagtcccagtgtctgctggggacgttcttcacctgccttgtgatcctgtttgcctgtgaggtggctgcaggcatctggggcttcgtaaacaaagaccagatcgccaaggatgtgaagcagttctatgaccaggcccttcagcaagctgtgatggatgatgatgccaacaatgccaaggctgtggtgaagactttccatgagacgctcaactgttgtggctccaacgcactgaccacactgactaccaccatactgaggaacagcctgtgtccctcaggcggcaacatactcacccccttactgcagcaagattgtcatcagaaaatcgatgagctcttctctgggaagctgtacctcattggaattgcagccattgtggtagctgtcattatgatctttgagatgattctgagcatggtgctgtgctgtggcatccggaacagctccgtgtactga

SEQ ID NO: 19 - protein, 306 aa, Mus musculus
MACNCQLMQDTPLLKFPCPRLILLFVLLIRLSQVSSDVDEQLSKSVKDKVLLPCRYNSPHEDESEDRIYWQKHDKVVLSVIAGKLKVWPEYKNRTLYDNTTYSLIILGLVLSDRGTYSCVVQKKERGTYEVKHLALVKLSIKADFSTPNITESGNPSADTKRITCFASGGFPKPRFSWLENGRELPGINTTISQDPESELYTISSQLDFNTTRNHTIKCLIKYGDAHVSEDFTWEKPPEDPPDSKNTLVLFGAGFGAVITVVVIVVIIKCFCKHRSCFRRNEASRETNNSLTFGPEEALAEQTVFL

SEQ ID NO: 20 - DNA, 921 bp, Mus musculus
atggcttgcaattgtcagttgatgcaggatacaccactcctcaagtttccatgtccaaggctcattcttctctttgtgctgctgattcgtctttcacaagtgtcttcagatgttgatgaacaactgtccaagtcagtgaaagataaggtattgctgccttgccgttacaactctcctcatgaagatgagtctgaagaccgaatctactggcaaaaacatgacaaagtggtgctgtctgtcattgctgggaaactaaaagtgtggcccgagtataagaaccggactttatatgacaacactacctactctcttatcatcctgggcctggtcctttcagaccggggcacatacagctgtgtcgttcaaaagaaggaaagaggaacgtatgaagttaaacacttggctttagtaaagttgtccatcaaagctgacttctctacccccaacataactgagtctggaaacccatctgcagacactaaaaggattacctgctttgcttccgggggtttcccaaagcctcgcttctcttggttggaaaatggaagagaattacctggcatcaatacgacaatttcccaggatcctgaatctgaattgtacaccattagtagccaactagatttcaatacgactcgcaaccacaccattaagtgtctcattaaatatggagatgctcacgtgtcagaggacttcacctgggaaaaacccccagaagaccctcctgatagcaagaacacacttgtgctctttggggcaggattcggcgcagtaataacagtcgtcgtcatcgttgtcatcatcaaatgcttctgtaagcacagaagctgtttcagaagaaatgaggcaagcagagaaacaaacaacagccttaccttcgggcctgaagaagcattagctgaacagaccgtcttcctttag

SEQ ID NO: 21 - protein, 226 aa, Mus musculus
MPVKGGSKCIKYLLFGFNFIFWLAGIAVLAIGLWLRFDSQTKSIFEQENNHSSFYTGVYILIGAGALMMLVGFLGCCGAVQESQCMLGLFFGFLLVIFAIEIAAAVWGYTHKDEVIKELQEFYKDTYQKLRSKDEPQRETLKAIHMALDCCGIAGPLEQFISDTCPKKQLLESFQVKPCPEAISEVFNNKFHIIGAVGIGIAVVMIFGMIFSMILCCAIRRSREMV

SEQ ID NO: 22 - DNA, 681 bp, Mus musculus
atgccggtcaaaggaggtagcaagtgcatcaaatacctgctcttcggatttaacttcatcttctggctcgctggcattgcagtgcttgctattggactatggctccgattcgactctcagaccaagagcatcttcgagcaagagaataaccattccagtttctacacaggagtgtacattctgattggagccggggccctcatgatgctggttggtttcctgggctgctgtggagctgtacaagagtcccagtgcatgctgggattgttcttcgggttcctcttggtgatattcgccattgagatagccgccgccgtctggggctatacccacaaggatgaggtgattaaagaactccaggagttttacaaggacacctaccaaaagttacggagcaaggatgaaccccagcgggaaacactcaaagccatccatatggcgttggactgctgtggcatagctggtcctttggagcagtttatctcggacacctgccccaagaaacagcttttggaaagtttccaggttaagccctgccctgaagccatcagtgaggtcttcaacaacaagttccacatcattggagcagtgggtatcggcatcgccgtggtgatgatcttcggcatgatcttcagcatgatcctgtgctgcgccatccgcaggagccgagaaatggtctag

SEQ ID NO: 23 - protein, 532 aa, Artificial Sequence
  peptide sequence derived from mus musculus
MACNCQLMQDTPLLKFPCPRLILLFVLLIRLSQVSSDVDEQLSKSVKDKVLLPCRYNSPHEDESEDRIYWQKHDKVVLSVIAGKLKVWPEYKNRTLYDNTTYSLIILGLVLSDRGTYSCVVQKKERGTYEVKHLALVKLSIKADFSTPNITESGNPSADTKRITCFASGGFPKPRFSWLENGRELPGINTTISQDPESELYTISSQLDFNTTRNHTIKCLIKYGDAHVSEDFTWEKPPEDPPDSKNTLVLFGAGFGAVITVVVIVVIIKCFCKHRSCFRRNEASRETNNSLTFGPEEALAEQTVFLMPVKGGSKCIKYLLFGFNFIFWLAGIAVLAIGLWLRFDSQTKSIFEQENNHSSFYTGVYILIGAGALMMLVGFLGCCGAVQESQCMLGLFFGFLLVIFAIEIAAAVWGYTHKDEVIKELQEFYKDTYQKLRSKDEPQRETLKAIHMALDCCGIAGPLEQFISDTCPKKQLLESFQVKPCPEAISEVFNNKFHIIGAVGIGIAVVMIFGMIFSMILCCAIRRSREMV

SEQ ID NO: 24 - DNA, 1599 bp, Artificial Sequence
  DNA sequence derived from mus musculus
atggcttgcaattgtcagttgatgcaggatacaccactcctcaagtttccatgtccaaggctcattcttctctttgtgctgctgattcgtctttcacaagtgtcttcagatgttgatgaacaactgtccaagtcagtgaaagataaggtattgctgccttgccgttacaactctcctcatgaagatgagtctgaagaccgaatctactggcaaaaacatgacaaagtggtgctgtctgtcattgctgggaaactaaaagtgtggcccgagtataagaaccggactttatatgacaacactacctactctcttatcatcctgggcctggtcctttcagaccggggcacatacagctgtgtcgttcaaaagaaggaaagaggaacgtatgaagttaaacacttggctttagtaaagttgtccatcaaagctgacttctctacccccaacataactgagtctggaaacccatctgcagacactaaaaggattacctgctttgcttccgggggtttcccaaagcctcgcttctcttggttggaaaatggaagagaattacctggcatcaatacgacaatttcccaggatcctgaatctgaattgtacaccattagtagccaactagatttcaatacgactcgcaaccacaccattaagtgtctcattaaatatggagatgctcacgtgtcagaggacttcacctgggaaaaacccccagaagaccctcctgatagcaagaacacacttgtgctctttggggcaggattcggcgcagtaataacagtcgtcgtcatcgttgtcatcatcaaatgcttctgtaagcacagaagctgtttcagaagaaatgaggcaagcagagaaacaaacaacagccttaccttcgggcctgaagaagcattagctgaacagaccgtcttccttatgccggtcaaaggaggtagcaagtgcatcaaatacctgctcttcggatttaacttcatcttctggctcgctggcattgcagtgcttgctattggactatggctccgattcgactctcagaccaagagcatcttcgagcaagagaataaccattccagtttctacacaggagtgtacattctgattggagccggggccctcatgatgctggttggtttcctgggctgctgtggagctgtacaagagtcccagtgcatgctgggattgttcttcgggttcctcttggtgatattcgccattgagatagccgccgccgtctggggctatacccacaaggatgaggtgattaaagaactccaggagttttacaaggacacctaccaaaagttacggagcaaggatgaaccccagcgggaaacactcaaagccatccatatggcgttggactgctgtggcatagctggtcctttggagcagtttatctcggacacctgccccaagaaacagcttttggaaagtttccaggttaagccctgccctgaagccatcagtgaggtcttcaacaacaagttccacatcattggagcagtgggtatcggcatcgccgtggtgatgatcttcggcatgatcttcagcatgatcctgtgctgcgccatccgcaggagccgagaaatggtctag

SEQ ID NO: 25 - protein, 149 aa, Mus musculus
APTSSSTSSSTAEAQQQQQQQQQQQQHLEQLLMDLQELLSRMENYRNLKLPRMLTFKFYLPKQATELKDLQCLEDELGPLRHVLDLTQSKSFQLEDAENFISNIRVTVVKLKGSDNTFECQFDDESATVVDFLRRWIAFCQSIISTSPQ

SEQ ID NO: 26 - DNA, 447 bp, Mus musculus
gcacccacttcaagctccacttcaagctctacagcggaagcacagcagcagcagcagcagcagcagcagcagcagcagcacctggagcagctgttgatggacctacaggagctcctgagcaggatggagaattacaggaacctgaaactccccaggatgctcaccttcaaattttacttgcccaagcaggccacagaattgaaagatcttcagtgcctagaagatgaacttggacctctgcggcatgttctggatttgactcaaagcaaaagctttcaattggaagatgctgagaatttcatcagcaatatcagagtaactgttgtaaaactaaagggctctgacaacacatttgagtgccaattcgatgatgagtcagcaactgtggtggactttctgaggagatggatagccttctgtcaaagcatcatctcaacaagccctcaa

SEQ ID NO: 27 - protein, 238 aa, Mus musculus
MAVEGGMKCVKFLLYVLLLAFCACAVGLIAIGVAVQVVLKQAITHETTAGSLLPVVIIAVGAFLFLVAFVGCCGACKENYCLMITFAIFLSLIMLVEVAVAIAGYVFRDQVKSEFNKSFQQQMQNYLKDNKTATILDKLQKENNCCGASNYTDWENIPGMAKDRVPDSCCINITVGCGNDFKESTIHTQGCVETIAIWLRKNILLVAAAALGIAFVEVLGIIFSCCLVKSIRSGYEVM

SEQ ID NO: 28 - DNA, 717 bp, Mus musculus
atggcggtggaaggaggaatgaagtgtgtcaagtttttgctctacgttctcctgctggccttctgcgcctgtgcagtgggattgatcgccattggtgtagcggttcaggttgtcttgaagcaggccattacccatgagactactgctggctcgctgttgcctgtggtcatcattgcagtgggtgccttcctcttcctggtggcctttgtgggctgctgtggggcctgcaaggagaactactgtctcatgattacatttgccatcttcctgtctcttatcatgcttgtggaggtggctgtggccattgctggctatgtgtttagagaccaggtgaagtcagagtttaataaaagcttccagcagcagatgcagaattaccttaaagacaacaaaacagccactattttggacaaattgcagaaagaaaataactgctgtggagcttctaactacacagactgggaaaacatccccggcatggccaaggacagagtccccgattcttgctgcatcaacataactgtgggctgtgggaatgatttcaaggaatccactatccatacccagggctgcgtggagactatagcaatatggctaaggaagaacatactgctggtggctgcagcggccctgggcattgcttttgtggaggtcttgggaattatcttctcctgctgtctggtgaagagtattcgaagtggctatgaagtaatgtag

SEQ ID NO: 29 - protein, 5 aa, Artificial Sequence
  synthesized peptide sequence
GGGGS

SEQ ID NO: 30 - DNA, 15 bp, Artificial Sequence
  synthesized DNA sequence
ggaggaggaggaagc

SEQ ID NO: 31 - protein, 397 aa, Artificial Sequence
  peptide sequence derived from mus musculus
MAVEGGMKCVKFLLYVLLLAFCACAVGLIAIGVAVQVVLKQAITHETTAGSLLPVVIIAVGAFLFLVAFVGCCGACKENYCLMITFAIFLSLIMLVEVAVAIAGYVFRDQVKSEFNKSFQQQMQNYLKDNKTATILDKLQKENNCCGASNYTDWENIPGMAKDRVPDSCCGGGGSAPTSSSTSSSTAEAQQQQQQQQQQQQHLEQLLMDLQELLSRMENYRNLKLPRMLTFKFYLPKQATELKDLQCLEDELGPLRHVLDLTQSKSFQLEDAENFISNIRVTVVKLKGSDNTFECQFDDESATVVDFLRRWIAFCQSIISTSPQGGGGSINITVGCGNDFKESTIHTQGCVETIAIWLRKNILLVAAAALGIAFVEVLGIIFSCCLVKSIRSGYEVM

SEQ ID NO: 32 - DNA, 1194 bp, Artificial Sequence
  DNA sequence derived from mus musculus
atggcggtggaaggaggaatgaagtgtgtcaagtttttgctctacgttctcctgctggccttctgcgcctgtgcagtgggattgatcgccattggtgtagcggttcaggttgtcttgaagcaggccattacccatgagactactgctggctcgctgttgcctgtggtcatcattgcagtgggtgccttcctcttcctggtggcctttgtgggctgctgtggggcctgcaaggagaactactgtctcatgattacatttgccatcttcctgtctcttatcatgcttgtggaggtggctgtggccattgctggctatgtgtttagagaccaggtgaagtcagagtttaataaaagcttccagcagcagatgcagaattaccttaaagacaacaaaacagccactattttggacaaattgcagaaagaaaataactgctgtggagcttctaactacacagactgggaaaacatccccggcatggccaaggacagagtccccgattcttgctgcggaggaggaggaagcgcacccacttcaagctccacttcaagctctacagcggaagcacagcagcagcagcagcagcagcagcagcagcagcagcacctggagcagctgttgatggacctacaggagctcctgagcaggatggagaattacaggaacctgaaactccccaggatgctcaccttcaaattttacttgcccaagcaggccacagaattgaaagatcttcagtgcctagaagatgaacttggacctctgcggcatgttctggatttgactcaaagcaaaagctttcaattggaagatgctgagaatttcatcagcaatatcagagtaactgttgtaaaactaaagggctctgacaacacatttgagtgccaattcgatgatgagtcagcaactgtggtggactttctgaggagatggatagccttctgtcaaagcatcatctcaacaagccctcaaggaggaggaggaagcatcaacataactgtgggctgtgggaatgatttcaaggaatccactatccatacccagggctgcgtggagactatagcaatatggctaaggaagaacatactgctggtggctgcagcggccctgggcattgcttttgtggaggtcttgggaattatcttctcctgctgtctggtgaagagtattcgaagtggctatgaagtaatgtag

SEQ ID NO: 33 - protein, 27 aa, Mus musculus
MALQIPSLLLSAAVVVLMVLSSPGTEG

SEQ ID NO: 34 - DNA, 81 bp, Mus musculus
atggctctgcagatccccagcctcctcctctcggctgctgtggtggtgctgatggtgctgagcagcccagggactgagggc

SEQ ID NO: 35 - protein, 17 aa, Artificial Sequence
  peptide sequence derived from OVA
ISQAVHAAHAEINEAGR

SEQ ID NO: 36 - DNA, 51 bp, Artificial Sequence
  DNA sequence derived from OVA
atatctcaagctgtccatgcagcacatgcagaaatcaatgaagcaggcaga

SEQ ID NO: 37 - protein, 238 aa, Mus musculus
GDSERHFVYQFMGECYFTNGTQRIRYVTRYIYNREEYVRYDSDVGEHRAVTELGRPDAEYWNSQPEILERTRAELDTVCRHNYEGPETHTSLRRLEQPNVVISLSRTEALNHHNTLVCSVTDFYPAKIKVRWFRNGQEETVGVSSTQLIRNGDWTFQVLVMLEMTPRRGEVYTCHVEHPSLKSPITVEWRAQSESAWSKMLSGIGGCVLGVIFLGLGLFIRHRSQKGPRGPPPAGLLQ

SEQ ID NO: 38 - DNA, 714 bp, Mus musculus
ggagactccgaaaggcatttcgtgtaccagttcatgggcgagtgctacttcaccaacgggacgcagcgcatacgatatgtgaccagatacatctacaaccgggaggagtacgtgcgctacgacagcgacgtgggcgagcaccgcgcggtgaccgagctggggcggccagacgccgagtactggaacagccagccggagatcctggagcgaacgcgggccgagctggacacggtgtgcagacacaactacgaggggccggagacccacacctccctgcggcggcttgaacagcccaatgtcgtcatctccctgtccaggacagaggccctcaaccaccacaacactctggtctgctcagtgacagatttctacccagccaagatcaaagtgcgctggttccggaatggccaggaggagacggtgggggtctcatccacacagcttattaggaatggggactggaccttccaggtcctggtcatgctggagatgacccctcggcggggagaggtctacacctgtcacgtggagcatcccagcctgaagagccccatcactgtggagtggagggcacagtctgagtctgcctggagcaagatgttgagcggcatcgggggctgcgtgcttggggtgatcttcctcgggcttggccttttcatccgtcacaggagtcagaaaggacctcgaggccctcctccagcagggctcctgcag

SEQ ID NO: 39 - protein, 11 aa, Artificial Sequence
  synthesized peptide sequence
GGGGSGGGGSG

SEQ ID NO: 40 - DNA, 33 bp, Artificial Sequence
  synthesized DNA sequence
ggaggaggaggaagcggaggaggaggaagcgga

SEQ ID NO: 41 - protein, 293 aa, Artificial Sequence
  peptide sequence derived from OVA, mus musculus
MALQIPSLLLSAAVVVLMVLSSPGTEGISQAVHAAHAEINEAGRGGGGSGGGGSGGDSERHFVYQFMGECYFTNGTQRIRYVTRYIYNREEYVRYDSDVGEHRAVTELGRPDAEYWNSQPEILERTRAELDTVCRHNYEGPETHTSLRRLEQPNVVISLSRTEALNHHNTLVCSVTDFYPAKIKVRWFRNGQEETVGVSSTQLIRNGDWTFQVLVMLEMTPRRGEVYTCHVEHPSLKSPITVEWRAQSESAWSKMLSGIGGCVLGVIFLGLGLFIRHRSQKGPRGPPPAGLLQ

SEQ ID NO: 42 - DNA, 879 bp, Artificial Sequence
  DNA sequence derived from OVA, mus musculus
atggctctgcagatccccagcctcctcctctcggctgctgtggtggtgctgatggtgctgagcagcccagggactgagggcatatctcaagctgtccatgcagcacatgcagaaatcaatgaagcaggcagaggaggaggaggaagcggaggaggaggaagcggaggagactccgaaaggcatttcgtgtaccagttcatgggcgagtgctacttcaccaacgggacgcagcgcatacgatatgtgaccagatacatctacaaccgggaggagtacgtgcgctacgacagcgacgtgggcgagcaccgcgcggtgaccgagctggggcggccagacgccgagtactggaacagccagccggagatcctggagcgaacgcgggccgagctggacacggtgtgcagacacaactacgaggggccggagacccacacctccctgcggcggcttgaacagcccaatgtcgtcatctccctgtccaggacagaggccctcaaccaccacaacactctggtctgctcagtgacagatttctacccagccaagatcaaagtgcgctggttccggaatggccaggaggagacggtgggggtctcatccacacagcttattaggaatggggactggaccttccaggtcctggtcatgctggagatgacccctcggcggggagaggtctacacctgtcacgtggagcatcccagcctgaagagccccatcactgtggagtggagggcacagtctgagtctgcctggagcaagatgttgagcggcatcgggggctgcgtgcttggggtgatcttcctcgggcttggccttttcatccgtcacaggagtcagaaaggacctcgaggccctcctccagcagggctcctgcag

SEQ ID NO: 43 - protein, 529 aa, Artificial Sequence
  peptide sequence derived from OVA, mus musculus
MALQIPSLLLSAAVVVLMVLSSPGTEGISQAVHAAHAEINEAGRGGGGSGGGGSGGDSERHFVYQFMGECYFTNGTQRIRYVTRYIYNREEYVRYDSDVGEHRAVTELGRPDAEYWNSQPEILERTRAELDTVCRHNYEGPETHTSLRRLEQPNVVISLSRTEALNHHNTLVCSVTDFYPAKIKVRWFRNGQEETVGVSSTQLIRNGDWTFQVLVMLEMTPRRGEVYTCHVEHPSLKSPITVEWRAQSESAWSKMLSGIGGCVLGVIFLGLGLFIRHRSQKGPRGPPPAGLLQMGVEGCTKCIKYLLFVFNFVFWLAGGVILGVALWLRHDPQTTSLLYLELGNKPAPNTFYVGIYILIAVGAVMMFVGFLGCYGAIQESQCLLGTFFTCLVILFACEVAAGIWGFVNKDQIAKDVKQFYDQALQQAVMDDDANNAKAVVKTFHETLNCCGSNALTTLTTTILRNSLCPSGGNILTPLLQQDCHQKIDELFSGKLYLIGIAAIVVAVIMIFEMILSMVLCCGIRNSSVY

SEQ ID NO: 44 - DNA, 1590 bp, Artificial Sequence
  DNA sequence derived from OVA, mus musculus
atggctctgcagatccccagcctcctcctctcggctgctgtggtggtgctgatggtgctgagcagcccagggactgagggcatatctcaagctgtccatgcagcacatgcagaaatcaatgaagcaggcagaggaggaggaggaagcggaggaggaggaagcggaggagactccgaaaggcatttcgtgtaccagttcatgggcgagtgctacttcaccaacgggacgcagcgcatacgatatgtgaccagatacatctacaaccgggaggagtacgtgcgctacgacagcgacgtgggcgagcaccgcgcggtgaccgagctggggcggccagacgccgagtactggaacagccagccggagatcctggagcgaacgcgggccgagctggacacggtgtgcagacacaactacgaggggccggagacccacacctccctgcggcggcttgaacagcccaatgtcgtcatctccctgtccaggacagaggccctcaaccaccacaacactctggtctgctcagtgacagatttctacccagccaagatcaaagtgcgctggttccggaatggccaggaggagacggtgggggtctcatccacacagcttattaggaatggggactggaccttccaggtcctggtcatgctggagatgacccctcggcggggagaggtctacacctgtcacgtggagcatcccagcctgaagagccccatcactgtggagtggagggcacagtctgagtctgcctggagcaagatgttgagcggcatcgggggctgcgtgcttggggtgatcttcctcgggcttggccttttcatccgtcacaggagtcagaaaggacctcgaggccctcctccagcagggctcctgcagatgggggtggagggctgcaccaaatgcatcaaatacctgctcttcgtcttcaatttcgtcttctggctggctggaggcgtgatcctaggtgtagctctgtggttgcgtcatgatccacagaccaccagcctgctgtacctggaactgggaaacaaaccggcacccaacaccttctacgtgggcatctacattctcattgctgtgggagctgtgatgatgtttgtaggcttcctggggtgctatggggccatccaggagtcccagtgtctgctggggacgttcttcacctgccttgtgatcctgtttgcctgtgaggtggctgcaggcatctggggcttcgtaaacaaagaccagatcgccaaggatgtgaagcagttctatgaccaggcccttcagcaagctgtgatggatgatgatgccaacaatgccaaggctgtggtgaagactttccatgagacgctcaactgttgtggctccaacgcactgaccacactgactaccaccatactgaggaacagcctgtgtccctcaggcggcaacatactcacccccttactgcagcaagattgtcatcagaaaatcgatgagctcttctctgggaagctgtacctcattggaattgcagccattgtggtagctgtcattatgatctttgagatgattctgagcatggtgctgtgctgtggcatccggaacagctccgtgtactga

SEQ ID NO: 45 - protein, 256 aa, Mus musculus
MPRSRALILGVLALTTMLSLCGGEDDIEADHVGTYGISVYQSPGDIGQYTFEFDGDELFYVDLDKKETVWMLPEFGQLASFDPQGGLQNIAVVKHNLGVLTKRSNSTPATNEAPQATVFPKSPVLLGQPNTLICFVDNIFPPVINITWLRNSKSVADGVYETSFFVNRDYSFHKLSYLTFIPSDDDIYDCKVEHWGLEEPVLKHWEPEIPAPMSELTETVVCALGLSVGLVGIVVGTIFIIQGLRSGGTSRHPGPL

SEQ ID NO: 46 - DNA, 771 bp, Mus musculus
atgccgcgcagcagagctctgattctgggggtcctcgccctgaccaccatgctcagcctctgtggaggtgaagacgacattgaggccgaccacgtaggcacctatggtataagtgtatatcagtctcctggagacattggccagtacacatttgaatttgatggtgatgagttgttctatgtggacttggataagaaggagactgtctggatgcttcctgagtttggccaattggcaagctttgacccccaaggtggactgcaaaacatagctgtagtaaaacacaacttgggagtcttgactaagaggtcaaattccaccccagctaccaatgaggctcctcaagcgactgtgttccccaagtcccctgtgctgctgggtcagcccaacaccctcatctgctttgtggacaacatcttccctcctgtgatcaacatcacatggctcagaaatagcaagtcagtcgcagacggtgtttatgagaccagcttcttcgtcaaccgtgactattccttccacaagctgtcttatctcaccttcatcccttctgacgatgacatttatgactgcaaggtggaacactggggcctggaggagccggttctgaaacactgggaacctgagattccagcccccatgtcagagctgacagagactgtggtctgtgccctggggttgtctgtgggccttgtgggcatcgtggtgggcaccatcttcatcattcaaggcctgcgatcaggtggcacctccagacacccagggcctttatga

SEQ ID NO: 47 - protein, 390 aa, Artificial Sequence
  peptide sequence derived from mus musculus
MPPSGLRLLPLLLPLPWLLVLTPGRPAAGLSTSKTIDMELVKRKRIEAIRGQILSKLRLASPPSQGEVPPGPLPEAVLALYNSTRDRVAGESADPEPEPEADYYAKEVTRVLMVDRNNAIYEKTKDISHSIYMFFNTSDIREAVPEPPLLSRAELRLQRLKSSVEQHVELYQKYSNNSWRYLGNRLLTPTDTPEWLSFDVTGVVRQWLNQGDGIQGFRFSAHSSSDSKDNKLHVEINGISPKRRGDLGTIHDMNRPFLLLMATPLERAQHLHSSRHRRALDTNYCFSSTEKNCCVRQLYIDFRKDLGWKWIHEPKGYHANFCLGPCPYIWSLDTQYSKVLALYNQHNPGASASPCCVPQALEPLPIVYYVGRKPKVEQLSNMIVRSCKCS

SEQ ID NO: 48 - DNA, 1173 bp, Artificial Sequence
  DNA sequence derived from mus musculus
atgccgccctcggggctgcggctactgccgcttctgctcccactcccgtggcttctagtgctgacgcccgggaggccagccgcgggactctccacctctaagaccatcgacatggagctggtgaaacggaagcgcatcgaagccatccgtggccagatcctgtccaaactaaggctcgccagtcccccaagccagggggaggtaccgcccggcccgctgcccgaggcggtgctcgctttgtacaacagcacccgcgaccgggtggcaggcgagagcgccgacccagagccggagcccgaagcggactactatgctaaagaggtcacccgcgtgctaatggtggaccgcaacaacgccatctatgagaaaaccaaagacatctcacacagtatatatatgttcttcaatacgtcagacattcgggaagcagtgcccgaacccccattgctgtcccgtgcagagctgcgcttgcagagattaaaatcaagtgtggagcaacatgtggaactctaccagaaatatagcaacaattcctggcgttaccttggtaaccggctgctgacccccactgatacgcctgagtggctgtcttttgacgtcactggagttgtacggcagtggctgaaccaaggagacggaatacagggctttcgattcagcgctcactcttcttctgacagcaaagataacaaactccacgtggaaatcaacgggatcagccccaaacgtcggggcgacctgggcaccatccatgacatgaaccggcccttcctgctcctcatggccacccccctggaaagggcccagcacctgcacagctcacggcaccggagagccctggataccaactattgcttcagctccacagagaagaactgctgtgtgcggcagctgtacattgactttaggaaggacctgggttggaagtggatccacgagcccaagggctaccatgccaacttctgtctgggaccctgcccctatatttggagcctggacacacagtacagcaaggtccttgccctctacaaccaacacaacccgggcgcttcggcgtcaccgtgctgcgtgccgcaggctttggagccactgcccatcgtctactacgtgggtcgcaagcccaaggtggagcagttgtccaacatgattgtgcgctcctgcaagtgcagctga

SEQ ID NO: 49 - protein, 441 aa, Artificial Sequence
  peptide sequence derived from mus musculus
ASGDFCDSSLCLNGGTCLTGQDNDIYCLCPEGFTGLVCNETERGPCSPNPCYNDAKCLVTLDTQRGEIFTEYICQCPVGYSGIHCETETNYYNLDGEYMFTTAVPNTAVPTPAPTPDLSNNLASRCSTQLGMEGGAIADSQISASSVYMGFMGLQRWGPELARLYRTGIVNAWTASNYDSKPWIQVNLLRKMRVSGVMTQGASRAGRAEYLKTFKVAYSLDGRKFEFIQDESGGDKEFLGNLDNNSLKVNMFNPTLEAQYIKLYPVSCHRGCTLRFELLGCELHGCSEPLGLKNNTIPDSQMSASSSYKTWNLRAFGWYPHLGRLDNQGKINAWTAQSNSAKEWLQVDLGTQRQVTGIITQGARDFGHIQYVASYKVAHSDDGVQWTVYEEQGSSKVFQGNLDNNSHKKNIFEKPFMARYVRVLPVSWHNRITLRLELLGC

SEQ ID NO: 50 - DNA, 1326 bp, Artificial Sequence
  DNA sequence derived from mus musculus
gcgtctggtgacttctgtgactccagcctgtgcctgaacggtggcacctgcttgacgggccaagacaatgacatctactgcctctgccctgaaggcttcacaggccttgtgtgcaatgagactgagagaggaccatgctccccaaacccttgctacaatgatgccaaatgtctggtgactttggacacacagcgtggggaaatcttcaccgaatacatctgccagtgccctgtgggctactcgggcatccactgtgaaaccgagaccaactactacaacctggatggagaatacatgttcaccacagccgtccccaatactgccgtccccaccccggcccccacccccgatctttccaacaacctagcctcccgttgttctacacagctgggcatggaagggggcgccattgctgattcacagatttccgcctcgtctgtgtatatgggtttcatgggcttgcagcgctggggcccggagctggctcgtctgtaccgcacagggatcgtcaatgcctggacagccagcaactatgatagcaagccctggatccaggtgaaccttctgcggaagatgcgggtatcaggtgtgatgacgcagggtgccagccgtgccgggagggcggagtacctgaagaccttcaaggtggcttacagcctcgacggacgcaagtttgagttcatccaggatgaaagcggtggagacaaggagtttttgggtaacctggacaacaacagcctgaaggttaacatgttcaacccgactctggaggcacagtacataaagctgtaccctgtttcgtgccaccgcggctgcaccctccgcttcgagctcctgggctgtgagttgcacggatgttctgagcccctgggcctgaagaataacacaattcctgacagccagatgtcagcctccagcagctacaagacatggaacctgcgtgcttttggctggtacccccacttgggaaggctggataatcagggcaagatcaatgcctggacggctcagagcaacagtgccaaggaatggctgcaggttgacctgggcactcagaggcaagtgacaggaatcatcacccagggggcccgtgactttggccacatccagtatgtggcgtcctacaaggtagcccacagtgatgatggtgtgcagtggactgtatatgaggagcaaggaagcagcaaggtcttccagggcaacttggacaacaactcccacaagaagaacatcttcgagaaacccttcatggctcgctacgtgcgtgtccttccagtgtcctggcataaccgcatcaccctgcgcctggagctgctgggctgttaa

SEQ ID NO: 51 - protein, 836 aa, Artificial Sequence
  peptide sequence derived from mus musculus
MPPSGLRLLPLLLPLPWLLVLTPGRPAAGLSTSKTIDMELVKRKRIEAIRGQILSKLRLASPPSQGEVPPGPLPEAVLALYNSTRDRVAGESADPEPEPEADYYAKEVTRVLMVDRNNAIYEKTKDISHSIYMFFNTSDIREAVPEPPLLSRAELRLQRLKSSVEQHVELYQKYSNNSWRYLGNRLLTPTDTPEWLSFDVTGVVRQWLNQGDGIQGFRFSAHSSSDSKDNKLHVEINGISPKRRGDLGTIHDMNRPFLLLMATPLERAQHLHSSRHRRALDTNYCFSSTEKNCCVRQLYIDFRKDLGWKWIHEPKGYHANFCLGPCPYIWSLDTQYSKVLALYNQHNPGASASPCCVPQALEPLPIVYYVGRKPKVEQLSNMIVRSCKCSGGGGSASGDFCDSSLCLNGGTCLTGQDNDIYCLCPEGFTGLVCNETERGPCSPNPCYNDAKCLVTLDTQRGEIFTEYICQCPVGYSGIHCETETNYYNLDGEYMFTTAVPNTAVPTPAPTPDLSNNLASRCSTQLGMEGGAIADSQISASSVYMGFMGLQRWGPELARLYRTGIVNAWTASNYDSKPWIQVNLLRKMRVSGVMTQGASRAGRAEYLKTFKVAYSLDGRKFEFIQDESGGDKEFLGNLDNNSLKVNMFNPTLEAQYIKLYPVSCHRGCTLRFELLGCELHGCSEPLGLKNNTIPDSQMSASSSYKTWNLRAFGWYPHLGRLDNQGKINAWTAQSNSAKEWLQVDLGTQRQVTGIITQGARDFGHIQYVASYKVAHSDDGVQWTVYEEQGSSKVFQGNLDNNSHKKNIFEKPFMARYVRVLPVSWHNRITLRLELLGC

SEQ ID NO: 52 - DNA, 2511 bp, Artificial Sequence
  DNA sequence derived from mus musculus
atgccgccctcggggctgcggctactgccgcttctgctcccactcccgtggcttctagtgctgacgcccgggaggccagccgcgggactctccacctctaagaccatcgacatggagctggtgaaacggaagcgcatcgaagccatccgtggccagatcctgtccaaactaaggctcgccagtcccccaagccagggggaggtaccgcccggcccgctgcccgaggcggtgctcgctttgtacaacagcacccgcgaccgggtggcaggcgagagcgccgacccagagccggagcccgaagcggactactatgctaaagaggtcacccgcgtgctaatggtggaccgcaacaacgccatctatgagaaaaccaaagacatctcacacagtatatatatgttcttcaatacgtcagacattcgggaagcagtgcccgaacccccattgctgtcccgtgcagagctgcgcttgcagagattaaaatcaagtgtggagcaacatgtggaactctaccagaaatatagcaacaattcctggcgttaccttggtaaccggctgctgacccccactgatacgcctgagtggctgtcttttgacgtcactggagttgtacggcagtggctgaaccaaggagacggaatacagggctttcgattcagcgctcactcttcttctgacagcaaagataacaaactccacgtggaaatcaacgggatcagccccaaacgtcggggcgacctgggcaccatccatgacatgaaccggcccttcctgctcctcatggccacccccctggaaagggcccagcacctgcacagctcacggcaccggagagccctggataccaactattgcttcagctccacagagaagaactgctgtgtgcggcagctgtacattgactttaggaaggacctgggttggaagtggatccacgagcccaagggctaccatgccaacttctgtctgggaccctgcccctatatttggagcctggacacacagtacagcaaggtccttgccctctacaaccaacacaacccgggcgcttcggcgtcaccgtgctgcgtgccgcaggctttggagccactgcccatcgtctactacgtgggtcgcaagcccaaggtggagcagttgtccaacatgattgtgcgctcctgcaagtgcagcggaggaggaggaagcgcgtctggtgacttctgtgactccagcctgtgcctgaacggtggcacctgcttgacgggccaagacaatgacatctactgcctctgccctgaaggcttcacaggccttgtgtgcaatgagactgagagaggaccatgctccccaaacccttgctacaatgatgccaaatgtctggtgactttggacacacagcgtggggaaatcttcaccgaatacatctgccagtgccctgtgggctactcgggcatccactgtgaaaccgagaccaactactacaacctggatggagaatacatgttcaccacagccgtccccaatactgccgtccccaccccggcccccacccccgatctttccaacaacctagcctcccgttgttctacacagctgggcatggaagggggcgccattgctgattcacagatttccgcctcgtctgtgtatatgggtttcatgggcttgcagcgctggggcccggagctggctcgtctgtaccgcacagggatcgtcaatgcctggacagccagcaactatgatagcaagccctggatccaggtgaaccttctgcggaagatgcgggtatcaggtgtgatgacgcagggtgccagccgtgccgggagggcggagtacctgaagaccttcaaggtggcttacagcctcgacggacgcaagtttgagttcatccaggatgaaagcggtggagacaaggagtttttgggtaacctggacaacaacagcctgaaggttaacatgttcaacccgactctggaggcacagtacataaagctgtaccctgtttcgtgccaccgcggctgcaccctccgcttcgagctcctgggctgtgagttgcacggatgttctgagcccctgggcctgaagaataacacaattcctgacagccagatgtcagcctccagcagctacaagacatggaacctgcgtgcttttggctggtacccccacttgggaaggctggataatcagggcaagatcaatgcctggacggctcagagcaacagtgccaaggaatggctgcaggttgacctgggcactcagaggcaagtgacaggaatcatcacccagggggcccgtgactttggccacatccagtatgtggcgtcctacaaggtagcccacagtgatgatggtgtgcagtggactgtatatgaggagcaaggaagcagcaaggtcttccagggcaacttggacaacaactcccacaagaagaacatcttcgagaaacccttcatggctcgctacgtgcgtgtccttccagtgtcctggcataaccgcatcaccctgcgcctggagctgctgggctgttaa

SEQ ID NO: 53 - protein, 120 aa, Mus musculus
HIHGCDKNHLREIIGILNEVTGEGTPCTEMDVPNVLTATKNTTESELVCRASKVLRIFYLKHGKTPCLKKNSSVLMELQRLFRAFRCLDSSISCTMNESKSTSLKDFLESLKSIMQMDYS

SEQ ID NO: 54 - DNA, 363 bp, Mus musculus
catatccacggatgcgacaaaaatcacttgagagagatcatcggcattttgaacgaggtcacaggagaagggacgccatgcacggagatggatgtgccaaacgtcctcacagcaacgaagaacaccacagagagtgagctcgtctgtagggcttccaaggtgcttcgcatattttatttaaaacatgggaaaactccatgcttgaagaagaactctagtgttctcatggagctgcagagactctttcgggcttttcgatgcctggattcatcgataagctgcaccatgaatgagtccaagtccacatcactgaaagacttcctggaaagcctaaagagcatcatgcaaatggattactcgtag

SEQ ID NO: 55 - protein, 366 aa, Artificial Sequence
  peptide sequence derived from mus musculus
MGVEGCTKCIKYLLFVFNFVFWLAGGVILGVALWLRHDPQTTSLLYLELGNKPAPNTFYVGIYILIAVGAVMMFVGFLGCYGAIQESQCLLGTFFTCLVILFACEVAAGIWGFVNKDQIAKDVKQFYDQALQQAVMDDDANNAKAVVKTFHETLNCCGSNALTTLTTTILRNSLCPSGGGGSHIHGCDKNHLREIIGILNEVTGEGTPCTEMDVPNVLTATKNTTESELVCRASKVLRIFYLKHGKTPCLKKNSSVLMELQRLFRAFRCLDSSISCTMNESKSTSLKDFLESLKSIMQMDYSGGGGSGGNILTPLLQQDCHQKIDELFSGKLYLIGIAAIVVAVIMIFEMILSMVLCCGIRNSSVY

SEQ ID NO: 56 - DNA, 1101 bp, Artificial Sequence
  DNA sequence derived from mus musculus
atgggggtggagggctgcaccaaatgcatcaaatacctgctcttcgtcttcaatttcgtcttctggctggctggaggcgtgatcctaggtgtagctctgtggttgcgtcatgatccacagaccaccagcctgctgtacctggaactgggaaacaaaccggcacccaacaccttctacgtgggcatctacattctcattgctgtgggagctgtgatgatgtttgtaggcttcctggggtgctatggggccatccaggagtcccagtgtctgctggggacgttcttcacctgccttgtgatcctgtttgcctgtgaggtggctgcaggcatctggggcttcgtaaacaaagaccagatcgccaaggatgtgaagcagttctatgaccaggcccttcagcaagctgtgatggatgatgatgccaacaatgccaaggctgtggtgaagactttccatgagacgctcaactgttgtggctccaacgcactgaccacactgactaccaccatactgaggaacagcctgtgtccctcaggaggaggaggaagccatatccacggatgcgacaaaaatcacttgagagagatcatcggcattttgaacgaggtcacaggagaagggacgccatgcacggagatggatgtgccaaacgtcctcacagcaacgaagaacaccacagagagtgagctcgtctgtagggcttccaaggtgcttcgcatattttatttaaaacatgggaaaactccatgcttgaagaagaactctagtgttctcatggagctgcagagactctttcgggcttttcgatgcctggattcatcgataagctgcaccatgaatgagtccaagtccacatcactgaaagacttcctggaaagcctaaagagcatcatgcaaatggattactcgggaggaggaggaagcggcggcaacatactcacccccttactgcagcaagattgtcatcagaaaatcgatgagctcttctctgggaagctgtacctcattggaattgcagccattgtggtagctgtcattatgatctttgagatgattctgagcatggtgctgtgctgtggcatccggaacagctccgtgtactga

SEQ ID NO: 57 - protein, 170 aa, Mus musculus
MAVEGGMKCVKFLLYVLLLAFCACAVGLIAIGVAVQVVLKQAITHETTAGSLLPVVIIAVGAFLFLVAFVGCCGACKENYCLMITFAIFLSLIMLVEVAVAIAGYVFRDQVKSEFNKSFQQQMQNYLKDNKTATILDKLQKENNCCGASNYTDWENIPGMAKDRVPDSCC

SEQ ID NO: 58 - DNA, 510 bp, Mus musculus
atggcggtggaaggaggaatgaagtgtgtcaagtttttgctctacgttctcctgctggccttctgcgcctgtgcagtgggattgatcgccattggtgtagcggttcaggttgtcttgaagcaggccattacccatgagactactgctggctcgctgttgcctgtggtcatcattgcagtgggtgccttcctcttcctggtggcctttgtgggctgctgtggggcctgcaaggagaactactgtctcatgattacatttgccatcttcctgtctcttatcatgcttgtggaggtggctgtggccattgctggctatgtgtttagagaccaggtgaagtcagagtttaataaaagcttccagcagcagatgcagaattaccttaaagacaacaaaacagccactattttggacaaattgcagaaagaaaataactgctgtggagcttctaactacacagactgggaaaacatccccggcatggccaaggacagagtccccgattcttgctgc

SEQ ID NO: 59 - protein, 68 aa, Mus musculus
INITVGCGNDFKESTIHTQGCVETIAIWLRKNILLVAAAALGIAFVEVLGIIFSCCLVKSIRSGYEVM

SEQ ID NO: 60 - DNA, 207 bp, Mus musculus
atcaacataactgtgggctgtgggaatgatttcaaggaatccactatccatacccagggctgcgtggagactatagcaatatggctaaggaagaacatactgctggtggctgcagcggccctgggcattgcttttgtggaggtcttgggaattatcttctcctgctgtctggtgaagagtattcgaagtggctatgaagtaatgtag

SEQ ID NO: 61 - protein, 177 aa, Mus musculus
MGVEGCTKCIKYLLFVFNFVFWLAGGVILGVALWLRHDPQTTSLLYLELGNKPAPNTFYVGIYILIAVGAVMMFVGFLGCYGAIQESQCLLGTFFTCLVILFACEVAAGIWGFVNKDQIAKDVKQFYDQALQQAVMDDDANNAKAVVKTFHETLNCCGSNALTTLTTTILRNSLCPS

SEQ ID NO: 62 - DNA, 531 bp, Mus musculus
atgggggtggagggctgcaccaaatgcatcaaatacctgctcttcgtcttcaatttcgtcttctggctggctggaggcgtgatcctaggtgtagctctgtggttgcgtcatgatccacagaccaccagcctgctgtacctggaactgggaaacaaaccggcacccaacaccttctacgtgggcatctacattctcattgctgtgggagctgtgatgatgtttgtaggcttcctggggtgctatggggccatccaggagtcccagtgtctgctggggacgttcttcacctgccttgtgatcctgtttgcctgtgaggtggctgcaggcatctggggcttcgtaaacaaagaccagatcgccaaggatgtgaagcagttctatgaccaggcccttcagcaagctgtgatggatgatgatgccaacaatgccaaggctgtggtgaagactttccatgagacgctcaactgttgtggctccaacgcactgaccacactgactaccaccatactgaggaacagcctgtgtccctca

SEQ ID NO: 63 - protein, 59 aa, Mus musculus
GGNILTPLLQQDCHQKIDELFSGKLYLIGIAAIVVAVIMIFEMILSMVLCCGIRNSSVY

SEQ ID NO: 64 - DNA, 180 bp, Mus musculus
ggcggcaacatactcacccccttactgcagcaagattgtcatcagaaaatcgatgagctcttctctgggaagctgtacctcattggaattgcagccattgtggtagctgtcattatgatctttgagatgattctgagcatggtgctgtgctgtggcatccggaacagctccgtgtactga

SEQ ID NO: 65 - protein, 467 aa, Artificial Sequence
  peptide sequence derived from mus musculus
IQKTPQIQVYSRHPPENGKPNILNCYVTQFHPPHIEIQMLKNGKKIPKVEMSDMSFSKDWSFYILAHTEFTPTETDTYACRVKHASMAEPKTVYWDRDMGGGGSGGGGSGGGGSGGGGSGPHSLRYFVTAVSRPGLGEPRYMEVGYVDDTEFVRFDSDAENPRYEPRARWMEQEGPEYWERETQKAKGNEQSFRVDLRTLLGYYNQSKGGSHTIQVISGCEVGSDGRLLRGYQQYAYDGCDYIALNEDLKTWTAADMAALITKHKWEQAGEAERLRAYLEGTCVEWLRRYLKNGNATLLRTDSPKAHVTHHSRPEDKVTLRCWALGFYPADITLTWQLNGEELIQDMELVETRPAGDGTFQKWASVVVPLGKEQYYTCHVYHQGLPEPLTLRWEPPPSTVSNMATVAVLVVLGAAIVTGAVVAFVMKMRRRNTGGKGGDYALAPGSQTSDLSLPDCKVMVHDPHSLA

SEQ ID NO: 66 - DNA, 1401 bp, Artificial Sequence
  DNA sequence derived from mus musculus
atccagaaaacccctcaaattcaagtatactcacgccacccaccggagaatgggaagccgaacatactgaactgctacgtaacacagttccacccgcctcacattgaaatccaaatgctgaagaacgggaaaaaaattcctaaagtagagatgtcagatatgtccttcagcaaggactggtctttctatatcctggctcacactgaattcacccccactgagactgatacatacgcctgcagagttaagcatgccagtatggccgagcccaagaccgtctactgggatcgagacatgggggggggaggctccggtggaggggggtctggagggggggggtctggtggaggcggaagtggcccacactcgctgaggtatttcgtcaccgccgtgtcccggcccggcctcggggagccccggtacatggaagtcggctacgtggacgacacggagttcgtgcgcttcgacagcgacgcggagaatccgagatatgagccgcgggcgcggtggatggagcaggaggggcccgagtattgggagcgggagacacagaaagccaagggcaatgagcagagtttccgagtggacctgaggaccctgctcggctactacaaccagagcaagggcggctctcacactattcaggtgatctctggctgtgaagtggggtccgacgggcgactcctccgcgggtaccagcagtacgcctacgacggctgcgattacatcgccctgaacgaagacctgaaaacgtggacggcggcggacatggcggcgctgatcaccaaacacaagtgggagcaggctggtgaagcagagagactcagggcctacctggagggcacgtgcgtggagtggctccgcagatacctgaagaacgggaacgcgacgctgctgcgcacagattccccaaaggcccatgtgacccatcacagcagacctgaagataaagtcaccctgaggtgctgggccctgggcttctaccctgctgacatcaccctgacctggcagttgaatggggaggagctgatccaggacatggagcttgtggagaccaggcctgcaggggatggaaccttccagaagtgggcatctgtggtggtgcctcttgggaaggagcagtattacacatgccatgtgtaccatcaggggctgcctgagcccctcaccctgagatgggagcctcctccatccactgtctccaacatggcgaccgttgctgttctggttgtccttggagctgcaatagtcactggagctgtggtggcttttgtgatgaagatgagaaggagaaacacaggtggaaaaggaggggactatgctctggctccaggctcccagacctctgatctgtctctcccagattgtaaagtgatggttcatgaccctcattctctagcg

SEQ ID NO: 67 - protein, 269 aa, Mus musculus
VDEQLSKSVKDKVLLPCRYNSPHEDESEDRIYWQKHDKVVLSVIAGKLKVWPEYKNRTLYDNTTYSLIILGLVLSDRGTYSCVVQKKERGTYEVKHLALVKLSIKADFSTPNITESGNPSADTKRITCFASGGFPKPRFSWLENGRELPGINTTISQDPESELYTISSQLDFNTTRNHTIKCLIKYGDAHVSEDFTWEKPPEDPPDSKNTLVLFGAGFGAVITVVVIVVIIKCFCKHRSCFRRNEASRETNNSLTFGPEEALAEQTVFL

SEQ ID NO: 68 - DNA, 810 bp, Mus musculus
gttgatgaacaactgtccaagtcagtgaaagataaggtattgctgccttgccgttacaactctcctcatgaagatgagtctgaagaccgaatctactggcaaaaacatgacaaagtggtgctgtctgtcattgctgggaaactaaaagtgtggcccgagtataagaaccggactttatatgacaacactacctactctcttatcatcctgggcctggtcctttcagaccggggcacatacagctgtgtcgttcaaaagaaggaaagaggaacgtatgaagttaaacacttggctttagtaaagttgtccatcaaagctgacttctctacccccaacataactgagtctggaaacccatctgcagacactaaaaggattacctgctttgcttccgggggtttcccaaagcctcgcttctcttggttggaaaatggaagagaattacctggcatcaatacgacaatttcccaggatcctgaatctgaattgtacaccattagtagccaactagatttcaatacgactcgcaaccacaccattaagtgtctcattaaatatggagatgctcacgtgtcagaggacttcacctgggaaaaacccccagaagaccctcctgatagcaagaacacacttgtgctctttggggcaggattcggcgcagtaataacagtcgtcgtcatcgttgtcatcatcaaatgcttctgtaagcacagaagctgtttcagaagaaatgaggcaagcagagaaacaaacaacagccttaccttcgggcctgaagaagcattagctgaacagaccgtcttcctttag

SEQ ID NO: 69 - protein, 495 aa, Artificial Sequence
  amino acid sequence derived from mus musculus
VDEQLSKSVKDKVLLPCRYNSPHEDESEDRIYWQKHDKVVLSVIAGKLKVWPEYKNRTLYDNTTYSLIILGLVLSDRGTYSCVVQKKERGTYEVKHLALVKLSIKADFSTPNITESGNPSADTKRITCFASGGFPKPRFSWLENGRELPGINTTISQDPESELYTISSQLDFNTTRNHTIKCLIKYGDAHVSEDFTWEKPPEDPPDSKNTLVLFGAGFGAVITVVVIVVIIKCFCKHRSCFRRNEASRETNNSLTFGPEEALAEQTVFLMPVKGGSKCIKYLLFGFNFIFWLAGIAVLAIGLWLRFDSQTKSIFEQENNHSSFYTGVYILIGAGALMMLVGFLGCCGAVQESQCMLGLFFGFLLVIFAIEIAAAVWGYTHKDEVIKELQEFYKDTYQKLRSKDEPQRETLKAIHMALDCCGIAGPLEQFISDTCPKKQLLESFQVKPCPEAISEVFNNKFHIIGAVGIGIAVVMIFGMIFSMILCCAIRRSREMV

SEQ ID NO: 70 - DNA, 1488 bp, Artificial Sequence
  DNA sequence derived from mus musculus
gttgatgaacaactgtccaagtcagtgaaagataaggtattgctgccttgccgttacaactctcctcatgaagatgagtctgaagaccgaatctactggcaaaaacatgacaaagtggtgctgtctgtcattgctgggaaactaaaagtgtggcccgagtataagaaccggactttatatgacaacactacctactctcttatcatcctgggcctggtcctttcagaccggggcacatacagctgtgtcgttcaaaagaaggaaagaggaacgtatgaagttaaacacttggctttagtaaagttgtccatcaaagctgacttctctacccccaacataactgagtctggaaacccatctgcagacactaaaaggattacctgctttgcttccgggggtttcccaaagcctcgcttctcttggttggaaaatggaagagaattacctggcatcaatacgacaatttcccaggatcctgaatctgaattgtacaccattagtagccaactagatttcaatacgactcgcaaccacaccattaagtgtctcattaaatatggagatgctcacgtgtcagaggacttcacctgggaaaaacccccagaagaccctcctgatagcaagaacacacttgtgctctttggggcaggattcggcgcagtaataacagtcgtcgtcatcgttgtcatcatcaaatgcttctgtaagcacagaagctgtttcagaagaaatgaggcaagcagagaaacaaacaacagccttaccttcgggcctgaagaagcattagctgaacagaccgtcttccttatgccggtcaaaggaggtagcaagtgcatcaaatacctgctcttcggatttaacttcatcttctggctcgctggcattgcagtgcttgctattggactatggctccgattcgactctcagaccaagagcatcttcgagcaagagaataaccattccagtttctacacaggagtgtacattctgattggagccggggccctcatgatgctggttggtttcctgggctgctgtggagctgtacaagagtcccagtgcatgctgggattgttcttcgggttcctcttggtgatattcgccattgagatagccgccgccgtctggggctatacccacaaggatgaggtgattaaagaactccaggagttttacaaggacacctaccaaaagttacggagcaaggatgaaccccagcgggaaacactcaaagccatccatatggcgttggactgctgtggcatagctggtcctttggagcagtttatctcggacacctgccccaagaaacagcttttggaaagtttccaggttaagccctgccctgaagccatcagtgaggtcttcaacaacaagttccacatcattggagcagtgggtatcggcatcgccgtggtgatgatcttcggcatgatcttcagcatgatcctgtgctgcgccatccgcaggagccgagaaatggtctag

SEQ ID NO: 71 - protein, 233 aa, Mus musculus
EDDIEADHVGTYGISVYQSPGDIGQYTFEFDGDELFYVDLDKKETVWMLPEFGQLASFDPQGGLQNIAVVKHNLGVLTKRSNSTPATNEAPQATVFPKSPVLLGQPNTLICFVDNIFPPVINITWLRNSKSVADGVYETSFFVNRDYSFHKLSYLTFIPSDDDIYDCKVEHWGLEEPVLKHWEPEIPAPMSELTETVVCALGLSVGLVGIVVGTIFIIQGLRSGGTSRHPGPL

SEQ ID NO: 72 - DNA, 702 bp, Mus musculus
gaagacgacattgaggccgaccacgtaggcacctatggtataagtgtatatcagtctcctggagacattggccagtacacatttgaatttgatggtgatgagttgttctatgtggacttggataagaaggagactgtctggatgcttcctgagtttggccaattggcaagctttgacccccaaggtggactgcaaaacatagctgtagtaaaacacaacttgggagtcttgactaagaggtcaaattccaccccagctaccaatgaggctcctcaagcgactgtgttccccaagtcccctgtgctgctgggtcagcccaacaccctcatctgctttgtggacaacatcttccctcctgtgatcaacatcacatggctcagaaatagcaagtcagtcgcagacggtgtttatgagaccagcttcttcgtcaaccgtgactattccttccacaagctgtcttatctcaccttcatcccttctgacgatgacatttatgactgcaaggtggaacactggggcctggaggagccggttctgaaacactgggaacctgagattccagcccccatgtcagagctgacagagactgtggtctgtgccctggggttgtctgtgggccttgtgggcatcgtggtgggcaccatcttcatcattcaaggcctgcgatcaggtggcacctccagacacccagggcctttatga

SEQ ID NO: 73 - protein, 361 aa, Mus musculus
LSTSKTIDMELVKRKRIEAIRGQILSKLRLASPPSQGEVPPGPLPEAVLALYNSTRDRVAGESADPEPEPEADYYAKEVTRVLMVDRNNAIYEKTKDISHSIYMFFNTSDIREAVPEPPLLSRAELRLQRLKSSVEQHVELYQKYSNNSWRYLGNRLLTPTDTPEWLSFDVTGVVRQWLNQGDGIQGFRFSAHSSSDSKDNKLHVEINGISPKRRGDLGTIHDMNRPFLLLMATPLERAQHLHSSRHRRALDTNYCFSSTEKNCCVRQLYIDFRKDLGWKWIHEPKGYHANFCLGPCPYIWSLDTQYSKVLALYNQHNPGASASPCCVPQALEPLPIVYYVGRKPKVEQLSNMIVRSCKCS

SEQ ID NO: 74 - DNA, 1086 bp, Mus musculus
ctctccacctctaagaccatcgacatggagctggtgaaacggaagcgcatcgaagccatccgtggccagatcctgtccaaactaaggctcgccagtcccccaagccagggggaggtaccgcccggcccgctgcccgaggcggtgctcgctttgtacaacagcacccgcgaccgggtggcaggcgagagcgccgacccagagccggagcccgaagcggactactatgctaaagaggtcacccgcgtgctaatggtggaccgcaacaacgccatctatgagaaaaccaaagacatctcacacagtatatatatgttcttcaatacgtcagacattcgggaagcagtgcccgaacccccattgctgtcccgtgcagagctgcgcttgcagagattaaaatcaagtgtggagcaacatgtggaactctaccagaaatatagcaacaattcctggcgttaccttggtaaccggctgctgacccccactgatacgcctgagtggctgtcttttgacgtcactggagttgtacggcagtggctgaaccaaggagacggaatacagggctttcgattcagcgctcactcttcttctgacagcaaagataacaaactccacgtggaaatcaacgggatcagccccaaacgtcggggcgacctgggcaccatccatgacatgaaccggcccttcctgctcctcatggccacccccctggaaagggcccagcacctgcacagctcacggcaccggagagccctggataccaactattgcttcagctccacagagaagaactgctgtgtgcggcagctgtacattgactttaggaaggacctgggttggaagtggatccacgagcccaagggctaccatgccaacttctgtctgggaccctgcccctatatttggagcctggacacacagtacagcaaggtccttgccctctacaaccaacacaacccgggcgcttcggcgtcaccgtgctgcgtgccgcaggctttggagccactgcccatcgtctactacgtgggtcgcaagcccaaggtggagcagttgtccaacatgattgtgcgctcctgcaagtgcagctga

SEQ ID NO: 75 - protein, 807 aa, Artificial Sequence
  amino acid sequence derived from mus musculus
LSTSKTIDMELVKRKRIEAIRGQILSKLRLASPPSQGEVPPGPLPEAVLALYNSTRDRVAGESADPEPEPEADYYAKEVTRVLMVDRNNAIYEKTKDISHSIYMFFNTSDIREAVPEPPLLSRAELRLQRLKSSVEQHVELYQKYSNNSWRYLGNRLLTPTDTPEWLSFDVTGVVRQWLNQGDGIQGFRFSAHSSSDSKDNKLHVEINGISPKRRGDLGTIHDMNRPFLLLMATPLERAQHLHSSRHRRALDTNYCFSSTEKNCCVRQLYIDFRKDLGWKWIHEPKGYHANFCLGPCPYIWSLDTQYSKVLALYNQHNPGASASPCCVPQALEPLPIVYYVGRKPKVEQLSNMIVRSCKCSGGGGSASGDFCDSSLCLNGGTCLTGQDNDIYCLCPEGFTGLVCNETERGPCSPNPCYNDAKCLVTLDTQRGEIFTEYICQCPVGYSGIHCETETNYYNLDGEYMFTTAVPNTAVPTPAPTPDLSNNLASRCSTQLGMEGGAIADSQISASSVYMGFMGLQRWGPELARLYRTGIVNAWTASNYDSKPWIQVNLLRKMRVSGVMTQGASRAGRAEYLKTFKVAYSLDGRKFEFIQDESGGDKEFLGNLDNNSLKVNMFNPTLEAQYIKLYPVSCHRGCTLRFELLGCELHGCSEPLGLKNNTIPDSQMSASSSYKTWNLRAFGWYPHLGRLDNQGKINAWTAQSNSAKEWLQVDLGTQRQVTGIITQGARDFGHIQYVASYKVAHSDDGVQWTVYEEQGSSKVFQGNLDNNSHKKNIFEKPFMARYVRVLPVSWHNRITLRLELLGC

SEQ ID NO: 76 - DNA, 2424 bp, Artificial Sequence
  DNA sequence derived from mus musculus
ctctccacctctaagaccatcgacatggagctggtgaaacggaagcgcatcgaagccatccgtggccagatcctgtccaaactaaggctcgccagtcccccaagccagggggaggtaccgcccggcccgctgcccgaggcggtgctcgctttgtacaacagcacccgcgaccgggtggcaggcgagagcgccgacccagagccggagcccgaagcggactactatgctaaagaggtcacccgcgtgctaatggtggaccgcaacaacgccatctatgagaaaaccaaagacatctcacacagtatatatatgttcttcaatacgtcagacattcgggaagcagtgcccgaacccccattgctgtcccgtgcagagctgcgcttgcagagattaaaatcaagtgtggagcaacatgtggaactctaccagaaatatagcaacaattcctggcgttaccttggtaaccggctgctgacccccactgatacgcctgagtggctgtcttttgacgtcactggagttgtacggcagtggctgaaccaaggagacggaatacagggctttcgattcagcgctcactcttcttctgacagcaaagataacaaactccacgtggaaatcaacgggatcagccccaaacgtcggggcgacctgggcaccatccatgacatgaaccggcccttcctgctcctcatggccacccccctggaaagggcccagcacctgcacagctcacggcaccggagagccctggataccaactattgcttcagctccacagagaagaactgctgtgtgcggcagctgtacattgactttaggaaggacctgggttggaagtggatccacgagcccaagggctaccatgccaacttctgtctgggaccctgcccctatatttggagcctggacacacagtacagcaaggtccttgccctctacaaccaacacaacccgggcgcttcggcgtcaccgtgctgcgtgccgcaggctttggagccactgcccatcgtctactacgtgggtcgcaagcccaaggtggagcagttgtccaacatgattgtgcgctcctgcaagtgcagcggaggaggaggaagcgcgtctggtgacttctgtgactccagcctgtgcctgaacggtggcacctgcttgacgggccaagacaatgacatctactgcctctgccctgaaggcttcacaggccttgtgtgcaatgagactgagagaggaccatgctccccaaacccttgctacaatgatgccaaatgtctggtgactttggacacacagcgtggggaaatcttcaccgaatacatctgccagtgccctgtgggctactcgggcatccactgtgaaaccgagaccaactactacaacctggatggagaatacatgttcaccacagccgtccccaatactgccgtccccaccccggcccccacccccgatctttccaacaacctagcctcccgttgttctacacagctgggcatggaagggggcgccattgctgattcacagatttccgcctcgtctgtgtatatgggtttcatgggcttgcagcgctggggcccggagctggctcgtctgtaccgcacagggatcgtcaatgcctggacagccagcaactatgatagcaagccctggatccaggtgaaccttctgcggaagatgcgggtatcaggtgtgatgacgcagggtgccagccgtgccgggagggcggagtacctgaagaccttcaaggtggcttacagcctcgacggacgcaagtttgagttcatccaggatgaaagcggtggagacaaggagtttttgggtaacctggacaacaacagcctgaaggttaacatgttcaacccgactctggaggcacagtacataaagctgtaccctgtttcgtgccaccgcggctgcaccctccgcttcgagctcctgggctgtgagttgcacggatgttctgagcccctgggcctgaagaataacacaattcctgacagccagatgtcagcctccagcagctacaagacatggaacctgcgtgcttttggctggtacccccacttgggaaggctggataatcagggcaagatcaatgcctggacggctcagagcaacagtgccaaggaatggctgcaggttgacctgggcactcagaggcaagtgacaggaatcatcacccagggggcccgtgactttggccacatccagtatgtggcgtcctacaaggtagcccacagtgatgatggtgtgcagtggactgtatatgaggagcaaggaagcagcaaggtcttccagggcaacttggacaacaactcccacaagaagaacatcttcgagaaacccttcatggctcgctacgtgcgtgtccttccagtgtcctggcataaccgcatcaccctgcgcctggagctgctgggctgttaa

SEQ ID NO: 77 - protein, 17 aa, Artificial Sequence
  synthesized amino acid sequence
TSGGSGGTGGSGGTGGS

SEQ ID NO: 78 - DNA, 51 bp, Artificial Sequence
  synthesized DNA sequence
accagcggaggaagcggtggcacaggcgggtctggaggcaccggaggctca

SEQ ID NO: 79 - protein, 14 aa, Artificial Sequence
  synthesized amino acid sequence
NYHLENEVARLKKL

SEQ ID NO: 80 - DNA, 42 bp, Artificial Sequence
  synthesized DNA sequence
aattaccacctggagaacgaagtggccaggctgaagaaactc

SEQ ID NO: 81 - protein, 274 aa, Artificial Sequence
  amino acid sequence derived from mus musculus
MALPVTALLLPLALLLHAARPEQKLISEEDLDAVVTQESALTSSPGETVTLTCRSSTGAVTTSNYASWVQEKPDHLFTGLIGGTNNRAPGVPARFSGSLIGDKAALTITGAQTEDEAIYFCVLWYSDHWVFGGGTKLTVLGGGGGSGGGGSGGGGSGGGGSDVQLQESGPGLVAPSQSLSITCTVSGFLLTDYGVNWVRQSPGKGLEWLGVIWGDGITDYNSALKSRLSVTKDNSKSQVFLKMNSLQSGDSARYYCVTGLFDYWGQGTTLTVSS

SEQ ID NO: 82 - DNA, 822 bp, Artificial Sequence
  DNA sequence derived from mus musculus
atggccttaccagtgaccgccttgctcctgccgctggccttgctgctccacgccgccaggccggagcagaagctgatcagcgaggaggacctggacgccgttgtgacccaggaatccgctctgacctcttctccaggcgaaaccgtgactctgacttgccgtagtagcaccggggctgtgaccacatctaactatgccagttgggtccaggaaaaaccggatcacctgtttactggcctgattggcggcaccaacaatcgcgcaccgggtgtgcccgctcgtttcagcggttccctgattggggacaaggcagcactgactatcaccggcgcccagaccgaagatgaggcgatctatttttgcgtcctgtggtacagcgaccattgggtgttcgggggaggcaccaaactgacagtgctgggcggaggaggaggttcaggaggaggaggtagcgggggaggcggttccgggggaggcggttctgatgtgcagctgcaagaatccgggccaggactggttgcgccttctcagagtctgtcaattacatgtactgttagtggctttctgctgaccgactatggtgtgaactgggttcgtcagagcccaggcaagggtctggagtggctgggagtgatttggggggatggaatcacagactacaatagcgcactgaaatctcggctgagtgttaccaaagataacagcaagtcccaggtcttcctgaagatgaacagcctgcaaagcggcgactccgctcgctattactgcgttaccggactgtttgattattgggggcaggggacaactctgactgtttcctcc

SEQ ID NO: 83 - protein, 253 aa, Artificial Sequence
  amino acid sequence derived from mus musculus
EQKLISEEDLDAVVTQESALTSSPGETVTLTCRSSTGAVTTSNYASWVQEKPDHLFTGLIGGTNNRAPGVPARFSGSLIGDKAALTITGAQTEDEAIYFCVLWYSDHWVFGGGTKLTVLGGGGGSGGGGSGGGGSGGGGSDVQLQESGPGLVAPSQSLSITCTVSGFLLTDYGVNWVRQSPGKGLEWLGVIWGDGITDYNSALKSRLSVTKDNSKSQVFLKMNSLQSGDSARYYCVTGLFDYWGQGTTLTVSS

SEQ ID NO: 84 - DNA, 759 bp, Artificial Sequence
  DNA sequence derived from mus musculus
gagcagaagctgatcagcgaggaggacctggacgccgttgtgacccaggaatccgctctgacctcttctccaggcgaaaccgtgactctgacttgccgtagtagcaccggggctgtgaccacatctaactatgccagttgggtccaggaaaaaccggatcacctgtttactggcctgattggcggcaccaacaatcgcgcaccgggtgtgcccgctcgtttcagcggttccctgattggggacaaggcagcactgactatcaccggcgcccagaccgaagatgaggcgatctatttttgcgtcctgtggtacagcgaccattgggtgttcgggggaggcaccaaactgacagtgctgggcggaggaggaggttcaggaggaggaggtagcgggggaggcggttccgggggaggcggttctgatgtgcagctgcaagaatccgggccaggactggttgcgccttctcagagtctgtcaattacatgtactgttagtggctttctgctgaccgactatggtgtgaactgggttcgtcagagcccaggcaagggtctggagtggctgggagtgatttggggggatggaatcacagactacaatagcgcactgaaatctcggctgagtgttaccaaagataacagcaagtcccaggtcttcctgaagatgaacagcctgcaaagcggcgactccgctcgctattactgcgttaccggactgtttgattattgggggcaggggacaactctgactgtttcctcc

SEQ ID NO: 85 - protein, 220 aa, Mus musculus
KPQAPELRIFPKKMDAELGQKVDLVCEVLGSVSQGCSWLFQNSSSKLPQPTFVVYMASSHNKITWDEKLNSSKLFSAMRDTNNKYVLTLNKFSKENEGYYFCSVISNSVMYFSSVVPVLQKVNSTTTKPVLRTPSPVHPTGTSQPQRPEDCRPRGSVKGTGLDFACDIYIWAPLAGICVALLLSLIITLICYHRSRKRVCKCPRPLVRQEGKPRPSEKIV

SEQ ID NO: 86 - DNA, 660 bp, Mus musculus
aagccacaggcacccgaactccgaatctttccaaagaaaatggacgccgaacttggtcagaaggtggacctggtatgtgaagtgttggggtccgtttcgcaaggatgctcttggctcttccagaactccagctccaaactcccccagcccaccttcgttgtctatatggcttcatcccacaacaagataacgtgggacgagaagctgaattcgtcgaaactgttttctgccatgagggacacgaataataagtacgttctcaccctgaacaagttcagcaaggaaaacgaaggctactatttctgctcagtcatcagcaactcggtgatgtacttcagttctgtcgtgccagtccttcagaaagtgaactctactactaccaagccagtgctgcgaactccctcacctgtgcaccctaccgggacatctcagccccagagaccagaagattgtcggccccgtggctcagtgaaggggaccggattggacttcgcctgtgatatttacatctgggcacccttggccggaatctgcgtggcccttctgctgtccttgatcatcactctcatctgctaccacaggagccgaaagcgtgtttgcaaatgtcccaggccgctagtcagacaggaaggcaagcccagaccttcagagaaaattgtg

SEQ ID NO: 87 - protein, 730 aa, Artificial Sequence
  amion acid sequence derived from mus musculus
MALPVTALLLPLALLLHAARPEQKLISEEDLDAVVTQESALTSSPGETVTLTCRSSTGAVTTSNYASWVQEKPDHLFTGLIGGTNNRAPGVPARFSGSLIGDKAALTITGAQTEDEAIYFCVLWYSDHWVFGGGTKLTVLGGGGGSGGGGSGGGGSGGGGSDVQLQESGPGLVAPSQSLSITCTVSGFLLTDYGVNWVRQSPGKGLEWLGVIWGDGITDYNSALKSRLSVTKDNSKSQVFLKMNSLQSGDSARYYCVTGLFDYWGQGTTLTVSSKPQAPELRIFPKKMDAELGQKVDLVCEVLGSVSQGCSWLFQNSSSKLPQPTFVVYMASSHNKITWDEKLNSSKLFSAMRDTNNKYVLTLNKFSKENEGYYFCSVISNSVMYFSSVVPVLQKVNSTTTKPVLRTPSPVHPTGTSQPQRPEDCRPRGSVKGTGLDFACDIYIWAPLAGICVALLLSLIITLICYHRSRKRVCKCPRPLVRQEGKPRPSEKIVMGVEGCTKCIKYLLFVFNFVFWLAGGVILGVALWLRHDPQTTSLLYLELGNKPAPNTFYVGIYILIAVGAVMMFVGFLGCYGAIQESQCLLGTFFTCLVILFACEVAAGIWGFVNKDQIAKDVKQFYDQALQQAVMDDDANNAKAVVKTFHETLNCCGSNALTTLTTTILRNSLCPSGGNILTPLLQQDCHQKIDELFSGKLYLIGIAAIVVAVIMIFEMILSMVLCCGIRNSSVY

SEQ ID NO: 88 - DNA, 2193 bp, Artificial Sequence
  DNA sequence derived from mus musculus
atggccttaccagtgaccgccttgctcctgccgctggccttgctgctccacgccgccaggccggagcagaagctgatcagcgaggaggacctggacgccgttgtgacccaggaatccgctctgacctcttctccaggcgaaaccgtgactctgacttgccgtagtagcaccggggctgtgaccacatctaactatgccagttgggtccaggaaaaaccggatcacctgtttactggcctgattggcggcaccaacaatcgcgcaccgggtgtgcccgctcgtttcagcggttccctgattggggacaaggcagcactgactatcaccggcgcccagaccgaagatgaggcgatctatttttgcgtcctgtggtacagcgaccattgggtgttcgggggaggcaccaaactgacagtgctgggcggaggaggaggttcaggaggaggaggtagcgggggaggcggttccgggggaggcggttctgatgtgcagctgcaagaatccgggccaggactggttgcgccttctcagagtctgtcaattacatgtactgttagtggctttctgctgaccgactatggtgtgaactgggttcgtcagagcccaggcaagggtctggagtggctgggagtgatttggggggatggaatcacagactacaatagcgcactgaaatctcggctgagtgttaccaaagataacagcaagtcccaggtcttcctgaagatgaacagcctgcaaagcggcgactccgctcgctattactgcgttaccggactgtttgattattgggggcaggggacaactctgactgtttcctccaagccacaggcacccgaactccgaatctttccaaagaaaatggacgccgaacttggtcagaaggtggacctggtatgtgaagtgttggggtccgtttcgcaaggatgctcttggctcttccagaactccagctccaaactcccccagcccaccttcgttgtctatatggcttcatcccacaacaagataacgtgggacgagaagctgaattcgtcgaaactgttttctgccatgagggacacgaataataagtacgttctcaccctgaacaagttcagcaaggaaaacgaaggctactatttctgctcagtcatcagcaactcggtgatgtacttcagttctgtcgtgccagtccttcagaaagtgaactctactactaccaagccagtgctgcgaactccctcacctgtgcaccctaccgggacatctcagccccagagaccagaagattgtcggccccgtggctcagtgaaggggaccggattggacttcgcctgtgatatttacatctgggcacccttggccggaatctgcgtggcccttctgctgtccttgatcatcactctcatctgctaccacaggagccgaaagcgtgtttgcaaatgtcccaggccgctagtcagacaggaaggcaagcccagaccttcagagaaaattgtgatgggggtggagggctgcaccaaatgcatcaaatacctgctcttcgtcttcaatttcgtcttctggctggctggaggcgtgatcctaggtgtagctctgtggttgcgtcatgatccacagaccaccagcctgctgtacctggaactgggaaacaaaccggcacccaacaccttctacgtgggcatctacattctcattgctgtgggagctgtgatgatgtttgtaggcttcctggggtgctatggggccatccaggagtcccagtgtctgctggggacgttcttcacctgccttgtgatcctgtttgcctgtgaggtggctgcaggcatctggggcttcgtaaacaaagaccagatcgccaaggatgtgaagcagttctatgaccaggcccttcagcaagctgtgatggatgatgatgccaacaatgccaaggctgtggtgaagactttccatgagacgctcaactgttgtggctccaacgcactgaccacactgactaccaccatactgaggaacagcctgtgtccctcaggcggcaacatactcacccccttactgcagcaagattgtcatcagaaaatcgatgagctcttctctgggaagctgtacctcattggaattgcagccattgtggtagctgtcattatgatctttgagatgattctgagcatggtgctgtgctgtggcatccggaacagctccgtgtactga

SEQ ID NO: 89 - protein, 709 aa, Artificial Sequence
  amino acid sequence derived from mus musculus
EQKLISEEDLDAVVTQESALTSSPGETVTLTCRSSTGAVTTSNYASWVQEKPDHLFTGLIGGTNNRAPGVPARFSGSLIGDKAALTITGAQTEDEAIYFCVLWYSDHWVFGGGTKLTVLGGGGGSGGGGSGGGGSGGGGSDVQLQESGPGLVAPSQSLSITCTVSGFLLTDYGVNWVRQSPGKGLEWLGVIWGDGITDYNSALKSRLSVTKDNSKSQVFLKMNSLQSGDSARYYCVTGLFDYWGQGTTLTVSSKPQAPELRIFPKKMDAELGQKVDLVCEVLGSVSQGCSWLFQNSSSKLPQPTFVVYMASSHNKITWDEKLNSSKLFSAMRDTNNKYVLTLNKFSKENEGYYFCSVISNSVMYFSSVVPVLQKVNSTTTKPVLRTPSPVHPTGTSQPQRPEDCRPRGSVKGTGLDFACDIYIWAPLAGICVALLLSLIITLICYHRSRKRVCKCPRPLVRQEGKPRPSEKIVMGVEGCTKCIKYLLFVFNFVFWLAGGVILGVALWLRHDPQTTSLLYLELGNKPAPNTFYVGIYILIAVGAVMMFVGFLGCYGAIQESQCLLGTFFTCLVILFACEVAAGIWGFVNKDQIAKDVKQFYDQALQQAVMDDDANNAKAVVKTFHETLNCCGSNALTTLTTTILRNSLCPSGGNILTPLLQQDCHQKIDELFSGKLYLIGIAAIVVAVIMIFEMILSMVLCCGIRNSSVY

SEQ ID NO: 90 - DNA, 2130 bp, Artificial Sequence
  DNA sequence derived from mus musculus
gagcagaagctgatcagcgaggaggacctggacgccgttgtgacccaggaatccgctctgacctcttctccaggcgaaaccgtgactctgacttgccgtagtagcaccggggctgtgaccacatctaactatgccagttgggtccaggaaaaaccggatcacctgtttactggcctgattggcggcaccaacaatcgcgcaccgggtgtgcccgctcgtttcagcggttccctgattggggacaaggcagcactgactatcaccggcgcccagaccgaagatgaggcgatctatttttgcgtcctgtggtacagcgaccattgggtgttcgggggaggcaccaaactgacagtgctgggcggaggaggaggttcaggaggaggaggtagcgggggaggcggttccgggggaggcggttctgatgtgcagctgcaagaatccgggccaggactggttgcgccttctcagagtctgtcaattacatgtactgttagtggctttctgctgaccgactatggtgtgaactgggttcgtcagagcccaggcaagggtctggagtggctgggagtgatttggggggatggaatcacagactacaatagcgcactgaaatctcggctgagtgttaccaaagataacagcaagtcccaggtcttcctgaagatgaacagcctgcaaagcggcgactccgctcgctattactgcgttaccggactgtttgattattgggggcaggggacaactctgactgtttcctccaagccacaggcacccgaactccgaatctttccaaagaaaatggacgccgaacttggtcagaaggtggacctggtatgtgaagtgttggggtccgtttcgcaaggatgctcttggctcttccagaactccagctccaaactcccccagcccaccttcgttgtctatatggcttcatcccacaacaagataacgtgggacgagaagctgaattcgtcgaaactgttttctgccatgagggacacgaataataagtacgttctcaccctgaacaagttcagcaaggaaaacgaaggctactatttctgctcagtcatcagcaactcggtgatgtacttcagttctgtcgtgccagtccttcagaaagtgaactctactactaccaagccagtgctgcgaactccctcacctgtgcaccctaccgggacatctcagccccagagaccagaagattgtcggccccgtggctcagtgaaggggaccggattggacttcgcctgtgatatttacatctgggcacccttggccggaatctgcgtggcccttctgctgtccttgatcatcactctcatctgctaccacaggagccgaaagcgtgtttgcaaatgtcccaggccgctagtcagacaggaaggcaagcccagaccttcagagaaaattgtgatgggggtggagggctgcaccaaatgcatcaaatacctgctcttcgtcttcaatttcgtcttctggctggctggaggcgtgatcctaggtgtagctctgtggttgcgtcatgatccacagaccaccagcctgctgtacctggaactgggaaacaaaccggcacccaacaccttctacgtgggcatctacattctcattgctgtgggagctgtgatgatgtttgtaggcttcctggggtgctatggggccatccaggagtcccagtgtctgctggggacgttcttcacctgccttgtgatcctgtttgcctgtgaggtggctgcaggcatctggggcttcgtaaacaaagaccagatcgccaaggatgtgaagcagttctatgaccaggcccttcagcaagctgtgatggatgatgatgccaacaatgccaaggctgtggtgaagactttccatgagacgctcaactgttgtggctccaacgcactgaccacactgactaccaccatactgaggaacagcctgtgtccctcaggcggcaacatactcacccccttactgcagcaagattgtcatcagaaaatcgatgagctcttctctgggaagctgtacctcattggaattgcagccattgtggtagctgtcattatgatctttgagatgattctgagcatggtgctgtgctgtggcatccggaacagctccgtgtactga

SEQ ID NO: 91 - protein, 732 aa, Artificial Sequence
  sc-Dimer-CD81-IL-12a
MALQIPSLLLSAAVVVLMVLSSPGTEGISQAVHAAHAEINEAGRGGGGSGGGGSGGDSERHFVYQFMGECYFTNGTQRIRYVTRYIYNREEYVRYDSDVGEHRAVTELGRPDAEYWNSQPEILERTRAELDTVCRHNYEGPETHTSLRRLEQPNVVISLSRTEALNHHNTLVCSVTDFYPAKIKVRWFRNGQEETVGVSSTQLIRNGDWTFQVLVMLEMTPRRGEVYTCHVEHPSLKSPITVEWRAQSESAWSKMLSGIGGCVLGVIFLGLGLFIRHRSQKGPRGPPPAGLLQMGVEGCTKCIKYLLFVFNFVFWLAGGVILGVALWLRHDPQTTSLLYLELGNKPAPNTFYVGIYILIAVGAVMMFVGFLGCYGAIQESQCLLGTFFTCLVILFACEVAAGIWGFVNKDQIAKDVKQFYDQALQQAVMDDDANNAKAVVKTFHETLNCCGSNALTTLTTTILRNSLCPSGGGGSRVIPVSGPARCLSQSRNLLKTTDDMVKTAREKLKHYSCTAEDIDHEDITRDQTSTLKTCLPLELHKNESCLATRETSSTTRGSCLPPQKTSLMMTLCLGSIYEDLKMYQTEFQAINAALQNHNHQQIILDKGMLVAIDELMQSLNHNGETLRQKPPVGEADPYRVKMKLCILLHAFSTRVVTINRVMGYLSSAGGGGSGGNILTPLLQQDCHQKIDELFSGKLYLIGIAAIVVAVIMIFEMILSMVLCCGIRNSSVY

SEQ ID NO: 92 - DNA, 2238 bp, Artificial Sequence
  sc-dimer-CD81-IL-12a
atggctctgcagatccccagcctcctcctctcggctgctgtggtggtgctgatggtgctgagcagcccagggactgagggcatatctcaagctgtccatgcagcacatgcagaaatcaatgaagcaggcagaggaggaggaggaagcggaggaggaggaagcggaggagactccgaaaggcatttcgtgtaccagttcatgggcgagtgctacttcaccaacgggacgcagcgcatacgatatgtgaccagatacatctacaaccgggaggagtacgtgcgctacgacagcgacgtgggcgagcaccgcgcggtgaccgagctggggcggccagacgccgagtactggaacagccagccggagatcctggagcgaacgcgggccgagctggacacggtgtgcagacacaactacgaggggccggagacccacacctccctgcggcggcttgaacagcccaatgtcgtcatctccctgtccaggacagaggccctcaaccaccacaacactctggtctgctcagtgacagatttctacccagccaagatcaaagtgcgctggttccggaatggccaggaggagacggtgggggtctcatccacacagcttattaggaatggggactggaccttccaggtcctggtcatgctggagatgacccctcggcggggagaggtctacacctgtcacgtggagcatcccagcctgaagagccccatcactgtggagtggagggcacagtctgagtctgcctggagcaagatgttgagcggcatcgggggctgcgtgcttggggtgatcttcctcgggcttggccttttcatccgtcacaggagtcagaaaggacctcgaggccctcctccagcagggctcctgcagatgggggtggagggctgcaccaaatgcatcaaatacctgctcttcgtcttcaatttcgtcttctggctggctggaggcgtgatcctaggtgtagctctgtggttgcgtcatgatccacagaccaccagcctgctgtacctggaactgggaaacaaaccggcacccaacaccttctacgtgggcatctacattctcattgctgtgggagctgtgatgatgtttgtaggcttcctggggtgctatggggccatccaggagtcccagtgtctgctggggacgttcttcacctgccttgtgatcctgtttgcctgtgaggtggctgcaggcatctggggcttcgtaaacaaagaccagatcgccaaggatgtgaagcagttctatgaccaggcccttcagcaagctgtgatggatgatgatgccaacaatgccaaggctgtggtgaagactttccatgagacgctcaactgttgtggctccaacgcactgaccacactgactaccaccatactgaggaacagcctgtgtccctcaggaggaggaggaagcagggtcattccagtctctggacctgccaggtgtcttagccagtcccgaaacctgctgaagaccacagatgacatggtgaagacggccagagaaaaactgaaacattattcctgcactgctgaagacatcgatcatgaagacatcacacgggaccaaaccagcacattgaagacctgtttaccactggaactacacaagaacgagagttgcctggctactagagagacttcttccacaacaagagggagctgcctgcccccacagaagacgtctttgatgatgaccctgtgccttggtagcatctatgaggacttgaagatgtaccagacagagttccaggccatcaacgcagcacttcagaatcacaaccatcagcagatcattctagacaagggcatgctggtggccatcgatgagctgatgcagtctctgaatcataatggcgagactctgcgccagaaacctcctgtgggagaagcagacccttacagagtgaaaatgaagctctgcatcctgcttcacgccttcagcacccgcgtcgtgaccatcaacagggtgatgggctatctgagctccgccggaggaggaggaagcggcggcaacatactcacccccttactgcagcaagattgtcatcagaaaatcgatgagctcttctctgggaagctgtacctcattggaattgcagccattgtggtagctgtcattatgatctttgagatgattctgagcatggtgctgtgctgtggcatccggaacagctccgtgtactgagtgctgtgctgtggcatccggaacagctccgtgtactga

SEQ ID NO: 93 - protein, 193 aa, Artificial Sequence
  Il-12a
RVIPVSGPARCLSQSRNLLKTTDDMVKTAREKLKHYSCTAEDIDHEDITRDQTSTLKTCLPLELHKNESCLATRETSSTTRGSCLPPQKTSLMMTLCLGSIYEDLKMYQTEFQAINAALQNHNHQQIILDKGMLVAIDELMQSLNHNGETLRQKPPVGEADPYRVKMKLCILLHAFSTRVVTINRVMGYLSSA

SEQ ID NO: 94 - DNA, 579 bp, Artificial Sequence
  IL-12a
agggtcattccagtctctggacctgccaggtgtcttagccagtcccgaaacctgctgaagaccacagatgacatggtgaagacggccagagaaaaactgaaacattattcctgcactgctgaagacatcgatcatgaagacatcacacgggaccaaaccagcacattgaagacctgtttaccactggaactacacaagaacgagagttgcctggctactagagagacttcttccacaacaagagggagctgcctgcccccacagaagacgtctttgatgatgaccctgtgccttggtagcatctatgaggacttgaagatgtaccagacagagttccaggccatcaacgcagcacttcagaatcacaaccatcagcagatcattctagacaagggcatgctggtggccatcgatgagctgatgcagtctctgaatcataatggcgagactctgcgccagaaacctcctgtgggagaagcagacccttacagagtgaaaatgaagctctgcatcctgcttcacgccttcagcacccgcgtcgtgaccatcaacagggtgatgggctatctgagctccgcc

SEQ ID NO: 95 - protein, 439 aa, Artificial Sequence
  CD81-IL12a
MGVEGCTKCIKYLLFVFNFVFWLAGGVILGVALWLRHDPQTTSLLYLELGNKPAPNTFYVGIYILIAVGAVMMFVGFLGCYGAIQESQCLLGTFFTCLVILFACEVAAGIWGFVNKDQIAKDVKQFYDQALQQAVMDDDANNAKAVVKTFHETLNCCGSNALTTLTTTILRNSLCPSGGGGSRVIPVSGPARCLSQSRNLLKTTDDMVKTAREKLKHYSCTAEDIDHEDITRDQTSTLKTCLPLELHKNESCLATRETSSTTRGSCLPPQKTSLMMTLCLGSIYEDLKMYQTEFQAINAALQNHNHQQIILDKGMLVAIDELMQSLNHNGETLRQKPPVGEADPYRVKMKLCILLHAFSTRVVTINRVMGYLSSAGGGGSGGNILTPLLQQDCHQKIDELFSGKLYLIGIAAIVVAVIMIFEMILSMVLCCGIRNSSVY

SEQ ID NO: 96 - DNA, 1320 bp, Artificial Sequence
  CD81-IL12a
atgggggtggagggctgcaccaaatgcatcaaatacctgctcttcgtcttcaatttcgtcttctggctggctggaggcgtgatcctaggtgtagctctgtggttgcgtcatgatccacagaccaccagcctgctgtacctggaactgggaaacaaaccggcacccaacaccttctacgtgggcatctacattctcattgctgtgggagctgtgatgatgtttgtaggcttcctggggtgctatggggccatccaggagtcccagtgtctgctggggacgttcttcacctgccttgtgatcctgtttgcctgtgaggtggctgcaggcatctggggcttcgtaaacaaagaccagatcgccaaggatgtgaagcagttctatgaccaggcccttcagcaagctgtgatggatgatgatgccaacaatgccaaggctgtggtgaagactttccatgagacgctcaactgttgtggctccaacgcactgaccacactgactaccaccatactgaggaacagcctgtgtccctcaggaggaggaggaagcagggtcattccagtctctggacctgccaggtgtcttagccagtcccgaaacctgctgaagaccacagatgacatggtgaagacggccagagaaaaactgaaacattattcctgcactgctgaagacatcgatcatgaagacatcacacgggaccaaaccagcacattgaagacctgtttaccactggaactacacaagaacgagagttgcctggctactagagagacttcttccacaacaagagggagctgcctgcccccacagaagacgtctttgatgatgaccctgtgccttggtagcatctatgaggacttgaagatgtaccagacagagttccaggccatcaacgcagcacttcagaatcacaaccatcagcagatcattctagacaagggcatgctggtggccatcgatgagctgatgcagtctctgaatcataatggcgagactctgcgccagaaacctcctgtgggagaagcagacccttacagagtgaaaatgaagctctgcatcctgcttcacgccttcagcacccgcgtcgtgaccatcaacagggtgatgggctatctgagctccgccggaggaggaggaagcggcggcaacatactcacccccttactgcagcaagattgtcatcagaaaatcgatgagctcttctctgggaagctgtacctcattggaattgcagccattgtggtagctgtcattatgatctttgagatgattctgagcatggtgctgtgctgtggcatccggaacagctccgtgtactga

SEQ ID NO: 97 - protein, 335 aa, Artificial Sequence
  IL-12b
MCPQKLTISWFAIVLLVSPLMAMWELEKDVYVVEVDWTPDAPGETVNLTCDTPEEDDITWTSDQRHGVIGSGKTLTITVKEFLDAGQYTCHKGGETLSHSHLLLHKKENGIWSTEILKNFKNKTFLKCEAPNYSGRFTCSWLVQRNMDLKFNIKSSSSSPDSRAVTCGMASLSAEKVTLDQRDYEKYSVSCQEDVTCPTAEETLPIELALEARQQNKYENYSTSFFIRDIIKPDPPKNLQMKPLKNSQVEVSWEYPDSWSTPHSYFSLKFFVRIQRKKEKMKETEEGCNQKGAFLVEKTSTEVQCKGGNVCVQAQDRYYNSSCSKWACVPCRVRS

SEQ ID NO: 98 - DNA, 1008 bp, Artificial Sequence
  IL-12b
atgtgtcctcagaagctaaccatctcctggtttgccatcgttttgctggtgtctccactcatggccatgtgggagctggagaaagacgtttatgttgtagaggtggactggactcccgatgcccctggagaaacagtgaacctcacctgtgacacgcctgaagaagatgacatcacctggacctcagaccagagacatggagtcataggctctggaaagaccctgaccatcactgtcaaagagtttctagatgctggccagtacacctgccacaaaggaggcgagactctgagccactcacatctgctgctccacaagaaggaaaatggaatttggtccactgaaattttaaaaaatttcaaaaacaagactttcctgaagtgtgaagcaccaaattactccggacggttcacgtgctcatggctggtgcaaagaaacatggacttgaagttcaacatcaagagcagtagcagttcccctgactctcgggcagtgacatgtggaatggcgtctctgtctgcagagaaggtcacactggaccaaagggactatgagaagtattcagtgtcctgccaggaggatgtcacctgcccaactgccgaggagaccctgcccattgaactggcgttggaagcacggcagcagaataaatatgagaactacagcaccagcttcttcatcagggacatcatcaaaccagacccgcccaagaacttgcagatgaagcctttgaagaactcacaggtggaggtcagctgggagtaccctgactcctggagcactccccattcctacttctccctcaagttctttgttcgaatccagcgcaagaaagaaaagatgaaggagacagaggaggggtgtaaccagaaaggtgcgttcctcgtagagaagacatctaccgaagtccaatgcaaaggcgggaatgtctgcgtgcaagctcaggatcgctattacaattcctcatgcagcaagtgggcatgtgttccctgcagggtccgatcctag

SEQ ID NO: 99 - protein, 187 aa, Artificial Sequence
  IL-6
FPTSQVRRGDFTEDTTPNRPVYTTSQVGGLITHVLWEIVEMRKELCNGNSDCMNNDDALAENNLKLPEIQRNDGCYQTGYNQEICLLKISSGLLEYHSYLEYMKNNLKDNKKDKARVLQRDTETLIHIFNQEVKDLHKIVLPTPISNALLTDKLESQKEWLRTKTIQFILKSLEEFLKVTLRSTRQT

SEQ ID NO: 100 - DNA, 561 bp, Artificial Sequence
  IL-6
ttccctacttcacaagtccggagaggagacttcacagaggataccactcccaacagacctgtctataccacttcacaagtcggaggcttaattacacatgttctctgggaaatcgtggaaatgagaaaagagttgtgcaatggcaattctgattgtatgaacaacgatgatgcacttgcagaaaacaatctgaaacttccagagatacaaagaaatgatggatgctaccaaactggatataatcaggaaatttgcctattgaaaatttcctctggtcttctggagtaccatagctacctggagtacatgaagaacaacttaaaagataacaagaaagacaaagccagagtccttcagagagatacagaaactctaattcatatcttcaaccaagaggtaaaagatttacataaaatagtccttcctaccccaatttccaatgctctcctaacagataagctggagtcacagaaggagtggctaaggaccaagaccatccaattcatcttgaaatcacttgaagaatttctaaaagtcactttgagatctactcggcaaacc

SEQ ID NO: 101 - protein, 433 aa, Artificial Sequence
  CD81-IL6
MGVEGCTKCIKYLLFVFNFVFWLAGGVILGVALWLRHDPQTTSLLYLELGNKPAPNTFYVGIYILIAVGAVMMFVGFLGCYGAIQESQCLLGTFFTCLVILFACEVAAGIWGFVNKDQIAKDVKQFYDQALQQAVMDDDANNAKAVVKTFHETLNCCGSNALTTLTTTILRNSLCPSGGGGSFPTSQVRRGDFTEDTTPNRPVYTTSQVGGLITHVLWEIVEMRKELCNGNSDCMNNDDALAENNLKLPEIQRNDGCYQTGYNQEICLLKISSGLLEYHSYLEYMKNNLKDNKKDKARVLQRDTETLIHIFNQEVKDLHKIVLPTPISNALLTDKLESQKEWLRTKTIQFILKSLEEFLKVTLRSTRQTGGGGSGGNILTPLLQQDCHQKIDELFSGKLYLIGIAAIVVAVIMIFEMILSMVLCCGIRNSSVY

SEQ ID NO: 102 - DNA, 1302 bp, Artificial Sequence
  CD81-IL6
atgggggtggagggctgcaccaaatgcatcaaatacctgctcttcgtcttcaatttcgtcttctggctggctggaggcgtgatcctaggtgtagctctgtggttgcgtcatgatccacagaccaccagcctgctgtacctggaactgggaaacaaaccggcacccaacaccttctacgtgggcatctacattctcattgctgtgggagctgtgatgatgtttgtaggcttcctggggtgctatggggccatccaggagtcccagtgtctgctggggacgttcttcacctgccttgtgatcctgtttgcctgtgaggtggctgcaggcatctggggcttcgtaaacaaagaccagatcgccaaggatgtgaagcagttctatgaccaggcccttcagcaagctgtgatggatgatgatgccaacaatgccaaggctgtggtgaagactttccatgagacgctcaactgttgtggctccaacgcactgaccacactgactaccaccatactgaggaacagcctgtgtccctcaggaggaggaggaagcttccctacttcacaagtccggagaggagacttcacagaggataccactcccaacagacctgtctataccacttcacaagtcggaggcttaattacacatgttctctgggaaatcgtggaaatgagaaaagagttgtgcaatggcaattctgattgtatgaacaacgatgatgcacttgcagaaaacaatctgaaacttccagagatacaaagaaatgatggatgctaccaaactggatataatcaggaaatttgcctattgaaaatttcctctggtcttctggagtaccatagctacctggagtacatgaagaacaacttaaaagataacaagaaagacaaagccagagtccttcagagagatacagaaactctaattcatatcttcaaccaagaggtaaaagatttacataaaatagtccttcctaccccaatttccaatgctctcctaacagataagctggagtcacagaaggagtggctaaggaccaagaccatccaattcatcttgaaatcacttgaagaatttctaaaagtcactttgagatctactcggcaaaccggaggaggaggaagcggcggcaacatactcacccccttactgcagcaagattgtcatcagaaaatcgatgagctcttctctgggaagctgtacctcattggaattgcagccattgtggtagctgtcattatgatctttgagatgattctgagcatggtgctgtgctgtggcatccggaacagctccgtgtactga

SEQ ID NO: 103 - protein, 288 aa, Artificial Sequence
  hCD80
MGHTRRQGTSPSKCPYLNFFQLLVLAGLSHFCSGVIHVTKEVKEVATLSCGHNVSVEELAQTRIYWQKEKKMVLTMMSGDMNIWPEYKNRTIFDITNNLSIVILALRPSDEGTYECVVLKYEKDAFKREHLAEVTLSVKADFPTPSISDFEIPTSNIRRIICSTSGGFPEPHLSWLENGEELNAINTTVSQDPETELYAVSSKLDFNMTTNHSFMCLIKYGHLRVNQTFNWNTTKQEHFPDNLLPSWAITLISVNGIFVICCLTYCFAPRCRERRRNERLRRESVRPV

SEQ ID NO: 104 - DNA, 864 bp, Artificial Sequence
  hCD81
atgggccacacacggaggcagggaacatcaccatccaagtgtccatacctcaatttctttcagctcttggtgctggctggtctttctcacttctgttcaggtgttatccacgtgaccaaggaagtgaaagaagtggcaacgctgtcctgtggtcacaatgtttctgttgaagagctggcacaaactcgcatctactggcaaaaggagaagaaaatggtgctgactatgatgtctggggacatgaatatatggcccgagtacaagaaccggaccatctttgatatcactaataacctctccattgtgatcctggctctgcgcccatctgacgagggcacatacgagtgtgttgttctgaagtatgaaaaagacgctttcaagcgggaacacctggctgaagtgacgttatcagtcaaagctgacttccctacacctagtatatctgactttgaaattccaacttctaatattagaaggataatttgctcaacctctggaggttttccagagcctcacctctcctggttggaaaatggagaagaattaaatgccatcaacacaacagtttcccaagatcctgaaactgagctctatgctgttagcagcaaactggatttcaatatgacaaccaaccacagcttcatgtgtctcatcaagtatggacatttaagagtgaatcagaccttcaactggaatacaaccaagcaagagcattttcctgataacctgctcccatcctgggccattaccttaatctcagtaaatggaatttttgtgatatgctgcctgacctactgctttgccccaagatgcagagagagaaggaggaatgagagattgagaagggaaagtgtacgccctgta

SEQ ID NO: 105 - protein, 228 aa, Artificial Sequence
  hCD9
MPVKGGTKCIKYLLFGFNFIFWLAGIAVLAIGLWLRFDSQTKSIFEQETNNNNSSFYTGVYILIGAGALMMLVGFLGCCGAVQESQCMLGLFFGFLLVIFAIEIAAAIWGYSHKDEVIKEVQEFYKDTYNKLKTKDEPQRETLKAIHYALNCCGLAGGVEQFISDICPKKDVLETFTVKSCPDAIKEVFDNKFHIIGAVGIGIAVVMIFGMIFSMILCCAIRRNREMV

SEQ ID NO: 106 - DNA, 687 bp, Artificial Sequence
  hCD9
atgccggtcaaaggaggcaccaagtgcatcaaatacctgctgttcggatttaacttcatcttctggcttgccgggattgctgtccttgccattggactatggctccgattcgactctcagaccaagagcatcttcgagcaagaaactaataataataattccagcttctacacaggagtctatattctgatcggagccggcgccctcatgatgctggtgggcttcctgggctgctgcggggctgtgcaggagtcccagtgcatgctgggactgttcttcggcttcctcttggtgatattcgccattgaaatagctgcggccatctggggatattcccacaaggatgaggtgattaaggaagtccaggagttttacaaggacacctacaacaagctgaaaaccaaggatgagccccagcgggaaacgctgaaagccatccactatgcgttgaactgctgtggtttggctgggggcgtggaacagtttatctcagacatctgccccaagaaggacgtactcgaaaccttcaccgtgaagtcctgtcctgatgccatcaaagaggtcttcgacaataaattccacatcatcggcgcagtgggcatcggcattgccgtggtcatgatatttggcatgatcttcagtatgatcttgtgctgtgctatccgcaggaaccgcgagatggtctag

SEQ ID NO: 107 - protein, 392 aa, Artificial Sequence
  hCD80-hCD9
MGHTRRQGTSPSKCPYLNFFQLLVLAGLSHFCSGVIHVTKEVKEVATLSCGHNVSVEELAQTRIYWQKEKKMVLTMMSGDMNIWPEYKNRTIFDITNNLSIVILALRPSDEGTYECVVLKYEKDAFKREHLAEVTLSVKADFPTPSISDFEIPTSNIRRIICSTSGGFPEPHLSWLENGEELNAINTTVSQDPETELYAVSSKLDFNMTTNHSFMCLIKYGHLRVNQTFNWNTTKQEHFPDNLLPSWAITLISVNGIFVICCLTYCFAPRCRERRRNERLRRESVRPVMPVKGGTKCIKYLLFGFNFIFWLAGIAVLAIGLWLRFDSQTKSIFEQETNNNNSSFYTGVYILIGAGALMMLVGFLGCCGAVQESQCMLGLFFGFLLVIFAIEI

SEQ ID NO: 108 - DNA, 1551 bp, Artificial Sequence
  hCD80-hCD9
atgggccacacacggaggcagggaacatcaccatccaagtgtccatacctcaatttctttcagctcttggtgctggctggtctttctcacttctgttcaggtgttatccacgtgaccaaggaagtgaaagaagtggcaacgctgtcctgtggtcacaatgtttctgttgaagagctggcacaaactcgcatctactggcaaaaggagaagaaaatggtgctgactatgatgtctggggacatgaatatatggcccgagtacaagaaccggaccatctttgatatcactaataacctctccattgtgatcctggctctgcgcccatctgacgagggcacatacgagtgtgttgttctgaagtatgaaaaagacgctttcaagcgggaacacctggctgaagtgacgttatcagtcaaagctgacttccctacacctagtatatctgactttgaaattccaacttctaatattagaaggataatttgctcaacctctggaggttttccagagcctcacctctcctggttggaaaatggagaagaattaaatgccatcaacacaacagtttcccaagatcctgaaactgagctctatgctgttagcagcaaactggatttcaatatgacaaccaaccacagcttcatgtgtctcatcaagtatggacatttaagagtgaatcagaccttcaactggaatacaaccaagcaagagcattttcctgataacctgctcccatcctgggccattaccttaatctcagtaaatggaatttttgtgatatgctgcctgacctactgctttgccccaagatgcagagagagaaggaggaatgagagattgagaagggaaagtgtacgccctgtaatgccggtcaaaggaggcaccaagtgcatcaaatacctgctgttcggatttaacttcatcttctggcttgccgggattgctgtccttgccattggactatggctccgattcgactctcagaccaagagcatcttcgagcaagaaactaataataataattccagcttctacacaggagtctatattctgatcggagccggcgccctcatgatgctggtgggcttcctgggctgctgcggggctgtgcaggagtcccagtgcatgctgggactgttcttcggcttcctcttggtgatattcgccattgaaatagctgcggccatctggggatattcccacaaggatgaggtgattaaggaagtccaggagttttacaaggacacctacaacaagctgaaaaccaaggatgagccccagcgggaaacgctgaaagccatccactatgcgttgaactgctgtggtttggctgggggcgtggaacagtttatctcagacatctgccccaagaaggacgtactcgaaaccttcaccgtgaagtcctgtcctgatgccatcaaagaggtcttcgacaataaattccacatcatcggcgcagtgggcatcggcattgccgtggtcatgatatttggcatgatcttcagtatgatcttgtgctgtgctatccgcaggaaccgcgagatggtctag

SEQ ID NO: 109 - protein, 133 aa, Artificial Sequence [sequence omitted]

SEQ ID NO: 110 - DNA, 399 bp, Artificial Sequence
  hIL-2
gcacctacttcaagttctacaaagaaaacacagctacaactggagcatttactgctggatttacagatgattttgaatggaattaataattacaagaatcccaaactcaccaggatgctcacatttaagttttacatgcccaagaaggccacagaactgaaacatcttcagtgtctagaagaagaactcaaacctctggaggaagtgctaaatttagctcaaagcaaaaactttcacttaagacccagggacttaatcagcaatatcaacgtaatagttctggaactaaagggatctgaaacaacattcatgtgtgaatatgctgatgagacagcaaccattgtagaatttctgaacagatggattaccttttgtcaaagcatcatctcaacactgact

SEQ ID NO: 111 - protein, 170 aa, Artificial Sequence
  hCD63 1-170
MAVEGGMKCVKFLLYVLLLAFCACAVGLIAVGVGAQLVLSQTIIQGATPGSLLPVVIIAVGVFLFLVAFVGCCGACKENYCLMITFAIFLSLIMLVEVAAAIAGYVFRDKVMSEFNNNFRQQMENYPKNNHTASILDRMQADFKCCGAANYTDWEKIPSMSKNRVPDSCC

SEQ ID NO: 112 - DNA, 510 bp, Artificial Sequence
  hCD63 1-170
atggcggtggaaggaggaatgaaatgtgtgaagttcttgctctacgtcctcctgctggccttttgcgcctgtgcagtgggactgattgccgtgggtgtcggggcacagcttgtcctgagtcagaccataatccagggggctacccctggctctctgttgccagtggtcatcatcgcagtgggtgtcttcctcttcctggtggcttttgtgggctgctgcggggcctgcaaggagaactattgtcttatgatcacgtttgccatctttctgtctcttatcatgttggtggaggtggccgcagccattgctggctatgtgtttagagataaggtgatgtcagagtttaataacaacttccggcagcagatggagaattacccgaaaaacaaccacactgcttcgatcctggacaggatgcaggcagattttaagtgctgtggggctgctaactacacagattgggagaaaatcccttccatgtcgaagaaccgagtccccgactcctgctgc

SEQ ID NO: 113 - protein, 68 aa, Artificial Sequence
  hCD63 171-238
INVTVGCGINFNEKAIHKEGCVEKIGGWLRKNVLVVAAAALGIAFVEVLGIVFACCLVKSIRSGYEVM

SEQ ID NO: 114 - DNA, 207 bp, Artificial Sequence
  hCD63 171-238
attaatgttactgtgggctgtgggattaatttcaacgagaaggcgatccataaggagggctgtgtggagaagattgggggctggctgaggaaaaatgtgctggtggtagctgcagcagcccttggaattgcttttgtcgaggttttgggaattgtctttgcctgctgcctcgtgaagagtatcagaagtggctacgaggtgatgtag

SEQ ID NO: 115 - protein, 381 aa, Artificial Sequence
  hCD63-IL2
MAVEGGMKCVKFLLYVLLLAFCACAVGLIAVGVGAQLVLSQTIIQGATPGSLLPVVIIAVGVFLFLVAFVGCCGACKENYCLMITFAIFLSLIMLVEVAAAIAGYVFRDKVMSEFNNNFRQQMENYPKNNHTASILDRMQADFKCCGAANYTDWEKIPSMSKNRVPDSCCGGGGSAPTSSSTKKTQLQLEHLLLDLQMILNGINNYKNPKLTRMLTFKFYMPKKATELKHLQCLEEELKPLEEVLNLAQSKNFHLRPRDLISNINVIVLELKGSETTFMCEYADETATIVEFLNRWITFCQSIISTLTGGGGSINVTVGCGINFNEKAIHKEGCVEKIGGWLRKNVLVVAAAALGIAFVEVLGIVFACCLVKSIRSGYEVM

SEQ ID NO: 116 - DNA, 1146 bp, Artificial Sequence
  hCD63-IL2
atggcggtggaaggaggaatgaaatgtgtgaagttcttgctctacgtcctcctgctggccttttgcgcctgtgcagtgggactgattgccgtgggtgtcggggcacagcttgtcctgagtcagaccataatccagggggctacccctggctctctgttgccagtggtcatcatcgcagtgggtgtcttcctcttcctggtggcttttgtgggctgctgcggggcctgcaaggagaactattgtcttatgatcacgtttgccatctttctgtctcttatcatgttggtggaggtggccgcagccattgctggctatgtgtttagagataaggtgatgtcagagtttaataacaacttccggcagcagatggagaattacccgaaaaacaaccacactgcttcgatcctggacaggatgcaggcagattttaagtgctgtggggctgctaactacacagattgggagaaaatcccttccatgtcgaagaaccgagtccccgactcctgctgcggaggaggaggaagcgcacctacttcaagttctacaaagaaaacacagctacaactggagcatttactgctggatttacagatgattttgaatggaattaataattacaagaatcccaaactcaccaggatgctcacatttaagttttacatgcccaagaaggccacagaactgaaacatcttcagtgtctagaagaagaactcaaacctctggaggaagtgctaaatttagctcaaagcaaaaactttcacttaagacccagggacttaatcagcaatatcaacgtaatagttctggaactaaagggatctgaaacaacattcatgtgtgaatatgctgatgagacagcaaccattgtagaatttctgaacagatggattaccttttgtcaaagcatcatctcaacactgactggaggaggaggaagcattaatgttactgtgggctgtgggattaatttcaacgagaaggcgatccataaggagggctgtgtggagaagattgggggctggctgaggaaaaatgtgctggtggtagctgcagcagcccttggaattgcttttgtcgaggttttgggaattgtctttgcctgctgcctcgtgaagagtatcagaagtggctacgaggtgatgtag

SEQ ID NO: 117 - protein, 20 aa, Artificial Sequence
  hb2mg signal
MSRSVALAVLALLSLSGLEA

SEQ ID NO: 118 - DNA, 60 bp, Artificial Sequence
  hb2mg signal
atgtctcgctccgtggccttagctgtgctcgcgctactctctctttctggcctggaggct

SEQ ID NO: 119 - protein, 9 aa, Artificial Sequence
  WT1
CYTWNQMNL

SEQ ID NO: 120 - DNA, 27 bp, Artificial Sequence
  WT1
tgctacacctggaaccagatgaacctg

SEQ ID NO: 121 - protein, 99 aa, Artificial Sequence [sequence omitted]

SEQ ID NO: 122 - DNA, 297 bp, Artificial Sequence
  hb2mg
atccagcgtactccaaagattcaggtttactcacgtcatccagcagagaatggaaagtcaaatttcctgaattgctatgtgtctgggtttcatccatccgacattgaagttgacttactgaagaatggagagagaattgaaaaagtggagcattcagacttgtctttcagcaaggactggtctttctatctcttgtactacactgaattcacccccactgaaaaagatgagtatgcctgccgtgtgaaccatgtgactttgtcacagcccaagatagttaagtgggatcgagacatg

SEQ ID NO: 123 - protein, 341 aa, Artificial Sequence
  hMHCIa
GSHSMRYFSTSVSRPGRGEPRFIAVGYVDDTQFVRFDSDAASQRMEPRAPWIEQEGPEYWDEETGKVKAHSQTDRENLRIALRYYNQSEAGSHTLQMMFGCDVGSDGRFLRGYHQYAYDGKDYIALKEDLRSWTAADMAAQITKRKWEAAHVAEQQRAYLEGTCVDGLRRYLENGKETLQRTDPPKTHMTHHPISDHEATLRCWALGFYPAEITLTWQRDGEDQTQDTELVETRPAGDGTFQKWAAVVVPSGEEQRYTCHVQHEGLPKPLTLRWEPSSQPTVPIVGIIAGLVLLGAVITGAVVAAVMWRRNSSDRKGGSYSQAASSDSAQGSDVSLTACKV

SEQ ID NO: 124 - DNA, 1023 bp, Artificial Sequence
  hMHCIa
ggctcccactccatgaggtatttctccacatccgtgtcccggcccggccgcggggagccccgcttcatcgccgtgggctacgtggacgacacgcagttcgtgcggttcgacagcgacgccgcgagccagaggatggagccgcgggcgccgtggatagagcaggaggggccggagtattgggacgaggagacagggaaagtgaaggcccactcacagactgaccgagagaacctgcggatcgcgctccgctactacaaccagagcgaggccggttctcacaccctccagatgatgtttggctgcgacgtggggtcggacgggcgcttcctccgcgggtaccaccagtacgcctacgacggcaaggattacatcgccctgaaagaggacctgcgctcttggaccgcggcggacatggcggctcagatcaccaagcgcaagtgggaggcggcccatgtggcggagcagcagagagcctacctggagggcacgtgcgtggacgggctccgcagatacctggagaacgggaaggagacgctgcagcgcacggacccccccaagacacatatgacccaccaccccatctctgaccatgaggccactctgagatgctgggccctgggcttctaccctgcggagatcacactgacctggcagcgggatggggaggaccagacccaggacacggagcttgtggagaccaggcctgcaggggatggaaccttccagaagtgggcagctgtggtggtaccttctggagaggagcagagatacacctgccatgtgcagcatgagggtctgcccaagcccctcaccctgagatgggagccatcttcccagcccaccgtccccatcgtgggcatcattgctggcctggttctccttggagctgtgatcactggagctgtggtcgctgctgtgatgtggaggaggaacagctcagatagaaaaggagggagctactctcaggctgcaagcagtgacagtgcccagggctctgatgtgtctctcacagcttgtaaagtg

SEQ ID NO: 125 - protein, 460 aa, Artificial Sequence
  hsMHCI
IQRTPKIQVYSRHPAENGKSNFLNCYVSGFHPSDIEVDLLKNGERIEKVEHSDLSFSKDWSFYLLYYTEFTPTEKDEYACRVNHVTLSQPKIVKWDRDMGGGGSGGGGSGGGGSGGGGSGSHSMRYFSTSVSRPGRGEPRFIAVGYVDDTQFVRFDSDAASQRMEPRAPWIEQEGPEYWDEETGKVKAHSQTDRENLRIALRYYNQSEAGSHTLQMMFGCDVGSDGRFLRGYHQYAYDGKDYIALKEDLRSWTAADMAAQITKRKWEAAHVAEQQRAYLEGTCVDGLRRYLENGKETLQRTDPPKTHMTHHPISDHEATLRCWALGFYPAEITLTWQRDGEDQTQDTELVETRPAGDGTFQKWAAVVVPSGEEQRYTCHVQHEGLPKPLTLRWEPSSQPTVPIVGIIAGLVLLGAVITGAVVAAVMWRRNSSDRKGGSYSQAASSDSAQGSDVSLTACKV

SEQ ID NO: 126 - DNA, 1380 bp, Artificial Sequence
  hsMHCI
atccagcgtactccaaagattcaggtttactcacgtcatccagcagagaatggaaagtcaaatttcctgaattgctatgtgtctgggtttcatccatccgacattgaagttgacttactgaagaatggagagagaattgaaaaagtggagcattcagacttgtctttcagcaaggactggtctttctatctcttgtactacactgaattcacccccactgaaaaagatgagtatgcctgccgtgtgaaccatgtgactttgtcacagcccaagatagttaagtgggatcgagacatgggggggggaggctccggtggaggggggtctggagggggggggtctggtggaggcggaagtggctcccactccatgaggtatttctccacatccgtgtcccggcccggccgcggggagccccgcttcatcgccgtgggctacgtggacgacacgcagttcgtgcggttcgacagcgacgccgcgagccagaggatggagccgcgggcgccgtggatagagcaggaggggccggagtattgggacgaggagacagggaaagtgaaggcccactcacagactgaccgagagaacctgcggatcgcgctccgctactacaaccagagcgaggccggttctcacaccctccagatgatgtttggctgcgacgtggggtcggacgggcgcttcctccgcgggtaccaccagtacgcctacgacggcaaggattacatcgccctgaaagaggacctgcgctcttggaccgcggcggacatggcggctcagatcaccaagcgcaagtgggaggcggcccatgtggcggagcagcagagagcctacctggagggcacgtgcgtggacgggctccgcagatacctggagaacgggaaggagacgctgcagcgcacggacccccccaagacacatatgacccaccaccccatctctgaccatgaggccactctgagatgctgggccctgggcttctaccctgcggagatcacactgacctggcagcgggatggggaggaccagacccaggacacggagcttgtggagaccaggcctgcaggggatggaaccttccagaagtgggcagctgtggtggtaccttctggagaggagcagagatacacctgccatgtgcagcatgagggtctgcccaagcccctcaccctgagatgggagccatcttcccagcccaccgtccccatcgtgggcatcattgctggcctggttctccttggagctgtgatcactggagctgtggtcgctgctgtgatgtggaggaggaacagctcagatagaaaaggagggagctactctcaggctgcaagcagtgacagtgcccagggctctgatgtgtctctcacagcttgtaaagtg

SEQ ID NO: 127 - protein, 504 aa, Artificial Sequence
  hsc-Trimer
MSRSVALAVLALLSLSGLEACYTWNQMNLGGGASGGGGSGGGGSIQRTPKIQVYSRHPAENGKSNFLNCYVSGFHPSDIEVDLLKNGERIEKVEHSDLSFSKDWSFYLLYYTEFTPTEKDEYACRVNHVTLSQPKIVKWDRDMGGGGSGGGGSGGGGSGGGGSGSHSMRYFSTSVSRPGRGEPRFIAVGYVDDTQFVRFDSDAASQRMEPRAPWIEQEGPEYWDEETGKVKAHSQTDRENLRIALRYYNQSEAGSHTLQMMFGCDVGSDGRFLRGYHQYAYDGKDYIALKEDLRSWTAADMAAQITKRKWEAAHVAEQQRAYLEGTCVDGLRRYLENGKETLQRTDPPKTHMTHHPISDHEATLRCWALGFYPAEITLTWQRDGEDQTQDTELVETRPAGDGTFQKWAAVVVPSGEEQRYTCHVQHEGLPKPLTLRWEPSSQPTVPIVGIIAGLVLLGAVITGAVVAAVMWRRNSSDRKGGSYSQAASSDSAQGSDVSLTACKV

SEQ ID NO: 128 - DNA, 1512 bp, Artificial Sequence
  hsc-Trimer
atgtctcgctccgtggccttagctgtgctcgcgctactctctctttctggcctggaggcttgctacacctggaaccagatgaacctgggcggaggtgcctctggcggtgggggcagcggtggagggggcagtatccagcgtactccaaagattcaggtttactcacgtcatccagcagagaatggaaagtcaaatttcctgaattgctatgtgtctgggtttcatccatccgacattgaagttgacttactgaagaatggagagagaattgaaaaagtggagcattcagacttgtctttcagcaaggactggtctttctatctcttgtactacactgaattcacccccactgaaaaagatgagtatgcctgccgtgtgaaccatgtgactttgtcacagcccaagatagttaagtgggatcgagacatgggggggggaggctccggtggaggggggtctggagggggggggtctggtggaggcggaagtggctcccactccatgaggtatttctccacatccgtgtcccggcccggccgcggggagccccgcttcatcgccgtgggctacgtggacgacacgcagttcgtgcggttcgacagcgacgccgcgagccagaggatggagccgcgggcgccgtggatagagcaggaggggccggagtattgggacgaggagacagggaaagtgaaggcccactcacagactgaccgagagaacctgcggatcgcgctccgctactacaaccagagcgaggccggttctcacaccctccagatgatgtttggctgcgacgtggggtcggacgggcgcttcctccgcgggtaccaccagtacgcctacgacggcaaggattacatcgccctgaaagaggacctgcgctcttggaccgcggcggacatggcggctcagatcaccaagcgcaagtgggaggcggcccatgtggcggagcagcagagagcctacctggagggcacgtgcgtggacgggctccgcagatacctggagaacgggaaggagacgctgcagcgcacggacccccccaagacacatatgacccaccaccccatctctgaccatgaggccactctgagatgctgggccctgggcttctaccctgcggagatcacactgacctggcagcgggatggggaggaccagacccaggacacggagcttgtggagaccaggcctgcaggggatggaaccttccagaagtgggcagctgtggtggtaccttctggagaggagcagagatacacctgccatgtgcagcatgagggtctgcccaagcccctcaccctgagatgggagccatcttcccagcccaccgtccccatcgtgggcatcattgctggcctggttctccttggagctgtgatcactggagctgtggtcgctgctgtgatgtggaggaggaacagctcagatagaaaaggagggagctactctcaggctgcaagcagtgacagtgcccagggctctgatgtgtctctcacagcttgtaaagtg

SEQ ID NO: 129 - protein, 236 aa, Artificial Sequence
  hCD81
MGVEGCTKCIKYLLFVFNFVFWLAGGVILGVALWLRHDPQTTNLLYLELGDKPAPNTFYVGIYILIAVGAVMMFVGFLGCYGAIQESQCLLGTFFTCLVILFACEVAAGIWGFVNKDQIAKDVKQFYDQALQQAVVDDDANNAKAVVKTFHETLDCCGSSTLTALTTSVLKNNLCPSGSNIISNLFKEDCHQKIDDLFSGKLYLIGIAAIVVAVIMIFEMILSMVLCCGIRNSSVY

SEQ ID NO: 130 - DNA, 711 bp, Artificial Sequence
  hCD81
atgggagtggagggctgcaccaagtgcatcaagtacctgctcttcgtcttcaatttcgtcttctggctggctggaggcgtgatcctgggtgtggccctgtggctccgccatgacccgcagaccaccaacctcctgtatctggagctgggagacaagcccgcgcccaacaccttctatgtaggcatctacatcctcatcgctgtgggcgctgtcatgatgttcgttggcttcctgggctgctacggggccatccaggaatcccagtgcctgctggggacgttcttcacctgcctggtcatcctgtttgcctgtgaggtggccgccggcatctggggctttgtcaacaaggaccagatcgccaaggatgtgaagcagttctatgaccaggccctacagcaggccgtggtggatgatgacgccaacaacgccaaggctgtggtgaagaccttccacgagacgcttgactgctgtggctccagcacactgactgctttgaccacctcagtgctcaagaacaatttgtgtccctcgggcagcaacatcatcagcaacctcttcaaggaggactgccaccagaagatcgatgacctcttctccgggaagctgtacctcatcggcattgctgccatcgtggtcgctgtgatcatgatcttcgagatgatcctgagcatggtgctgtgctgtggcatccggaacagctccgtgtactga

SEQ ID NO: 131 - protein, 740 aa, Artificial Sequence
  hsc-Trimer-CD81
MSRSVALAVLALLSLSGLEACYTWNQMNLGGGASGGGGSGGGGSIQRTPKIQVYSRHPAENGKSNFLNCYVSGFHPSDIEVDLLKNGERIEKVEHSDLSFSKDWSFYLLYYTEFTPTEKDEYACRVNHVTLSQPKIVKWDRDMGGGGSGGGGSGGGGSGGGGSGSHSMRYFSTSVSRPGRGEPRFIAVGYVDDTQFVRFDSDAASQRMEPRAPWIEQEGPEYWDEETGKVKAHSQTDRENLRIALRYYNQSEAGSHTLQMMFGCDVGSDGRFLRGYHQYAYDGKDYIALKEDLRSWTAADMAAQITKRKWEAAHVAEQQRAYLEGTCVDGLRRYLENGKETLQRTDPPKTHMTHHPISDHEATLRCWALGFYPAEITLTWQRDGEDQTQDTELVETRPAGDGTFQKWAAVVVPSGEEQRYTCHVQHEGLPKPLTLRWEPSSQPTVPIVGIIAGLVLLGAVITGAVVAAVMWRRNSSDRKGGSYSQAASSDSAQGSDVSLTACKVMGVEGCTKCIKYLLFVFNFVFWLAGGVILGVALWLRHDPQTTNLLYLELGDKPAPNTFYVGIYILIAVGAVMMFVGFLGCYGAIQESQCLLGTFFTCLVILFACEVAAGIWGFVNKDQIAKDVKQFYDQALQQAVVDDDANNAKAVVKTFHETLDCCGSSTLTALTTSVLKNNLCPSGSNIISNLFKEDCHQKIDDLFSGKLYLIGIAAIVVAVIMIFEMILSMVLCCGIRNSSVY

SEQ ID NO: 132 - DNA, 2223 bp, Artificial Sequence
  hsc-Trimer-CD81
atgtctcgctccgtggccttagctgtgctcgcgctactctctctttctggcctggaggcttgctacacctggaaccagatgaacctgggcggaggtgcctctggcggtgggggcagcggtggagggggcagtatccagcgtactccaaagattcaggtttactcacgtcatccagcagagaatggaaagtcaaatttcctgaattgctatgtgtctgggtttcatccatccgacattgaagttgacttactgaagaatggagagagaattgaaaaagtggagcattcagacttgtctttcagcaaggactggtctttctatctcttgtactacactgaattcacccccactgaaaaagatgagtatgcctgccgtgtgaaccatgtgactttgtcacagcccaagatagttaagtgggatcgagacatgggggggggaggctccggtggaggggggtctggagggggggggtctggtggaggcggaagtggctcccactccatgaggtatttctccacatccgtgtcccggcccggccgcggggagccccgcttcatcgccgtgggctacgtggacgacacgcagttcgtgcggttcgacagcgacgccgcgagccagaggatggagccgcgggcgccgtggatagagcaggaggggccggagtattgggacgaggagacagggaaagtgaaggcccactcacagactgaccgagagaacctgcggatcgcgctccgctactacaaccagagcgaggccggttctcacaccctccagatgatgtttggctgcgacgtggggtcggacgggcgcttcctccgcgggtaccaccagtacgcctacgacggcaaggattacatcgccctgaaagaggacctgcgctcttggaccgcggcggacatggcggctcagatcaccaagcgcaagtgggaggcggcccatgtggcggagcagcagagagcctacctggagggcacgtgcgtggacgggctccgcagatacctggagaacgggaaggagacgctgcagcgcacggacccccccaagacacatatgacccaccaccccatctctgaccatgaggccactctgagatgctgggccctgggcttctaccctgcggagatcacactgacctggcagcgggatggggaggaccagacccaggacacggagcttgtggagaccaggcctgcaggggatggaaccttccagaagtgggcagctgtggtggtaccttctggagaggagcagagatacacctgccatgtgcagcatgagggtctgcccaagcccctcaccctgagatgggagccatcttcccagcccaccgtccccatcgtgggcatcattgctggcctggttctccttggagctgtgatcactggagctgtggtcgctgctgtgatgtggaggaggaacagctcagatagaaaaggagggagctactctcaggctgcaagcagtgacagtgcccagggctctgatgtgtctctcacagcttgtaaagtgatgggagtggagggctgcaccaagtgcatcaagtacctgctcttcgtcttcaatttcgtcttctggctggctggaggcgtgatcctgggtgtggccctgtggctccgccatgacccgcagaccaccaacctcctgtatctggagctgggagacaagcccgcgcccaacaccttctatgtaggcatctacatcctcatcgctgtgggcgctgtcatgatgttcgttggcttcctgggctgctacggggccatccaggaatcccagtgcctgctggggacgttcttcacctgcctggtcatcctgtttgcctgtgaggtggccgccggcatctggggctttgtcaacaaggaccagatcgccaaggatgtgaagcagttctatgaccaggccctacagcaggccgtggtggatgatgacgccaacaacgccaaggctgtggtgaagaccttccacgagacgcttgactgctgtggctccagcacactgactgctttgaccacctcagtgctcaagaacaatttgtgtccctcgggcagcaacatcatcagcaacctcttcaaggaggactgccaccagaagatcgatgacctcttctccgggaagctgtacctcatcggcattgctgccatcgtggtcgctgtgatcatgatcttcgagatgatcctgagcatggtgctgtgctgtggcatccggaacagctccgtgtactga

SEQ ID NO: 133 - protein, 395 aa, Artificial Sequence
  CD81-IL-2
MGVEGCTKCIKYLLFVFNFVFWLAGGVILGVALWLRHDPQTTSLLYLELGNKPAPNTFYVGIYILIAVGAVMMFVGFLGCYGAIQESQCLLGTFFTCLVILFACEVAAGIWGFVNKDQIAKDVKQFYDQALQQAVMDDDANNAKAVVKTFHETLNCCGSNALTTLTTTILRNSLCPSGGGGSAPTSSSTSSSTAEAQQQQQQQQQQQQHLEQLLMDLQELLSRMENYRNLKLPRMLTFKFYLPKQATELKDLQCLEDELGPLRHVLDLTQSKSFQLEDAENFISNIRVTVVKLKGSDNTFECQFDDESATVVDFLRRWIAFCQSIISTSPQGGGGSGGNILTPLLQQDCHQKIDELFSGKLYLIGIAAIVVAVIMIFEMILSMVLCCGIRNSSVY

SEQ ID NO: 134 - DNA, 1188 bp, Artificial Sequence
  CD81-IL2
atgggggtggagggctgcaccaaatgcatcaaatacctgctcttcgtcttcaatttcgtcttctggctggctggaggcgtgatcctaggtgtagctctgtggttgcgtcatgatccacagaccaccagcctgctgtacctggaactgggaaacaaaccggcacccaacaccttctacgtgggcatctacattctcattgctgtgggagctgtgatgatgtttgtaggcttcctggggtgctatggggccatccaggagtcccagtgtctgctggggacgttcttcacctgccttgtgatcctgtttgcctgtgaggtggctgcaggcatctggggcttcgtaaacaaagaccagatcgccaaggatgtgaagcagttctatgaccaggcccttcagcaagctgtgatggatgatgatgccaacaatgccaaggctgtggtgaagactttccatgagacgctcaactgttgtggctccaacgcactgaccacactgactaccaccatactgaggaacagcctgtgtccctcaggaggaggaggaagcgcacccacttcaagctccacttcaagctctacagcggaagcacagcagcagcagcagcagcagcagcagcagcagcagcacctggagcagctgttgatggacctacaggagctcctgagcaggatggagaattacaggaacctgaaactccccaggatgctcaccttcaaattttacttgcccaagcaggccacagaattgaaagatcttcagtgcctagaagatgaacttggacctctgcggcatgttctggatttgactcaaagcaaaagctttcaattggaagatgctgagaatttcatcagcaatatcagagtaactgttgtaaaactaaagggctctgacaacacatttgagtgccaattcgatgatgagtcagcaactgtggtggactttctgaggagatggatagccttctgtcaaagcatcatctcaacaagccctcaaggaggaggaggaagcggcggcaacatactcacccccttactgcagcaagattgtcatcagaaaatcgatgagctcttctctgggaagctgtacctcattggaattgcagccattgtggtagctgtcattatgatctttgagatgattctgagcatggtgctgtgctgtggcatccggaacagctccgtgtactga

SEQ ID NO: 135 - protein, 905 aa, Artificial Sequence
  sc-Trimer-CD81-IL-2
MARSVTLVFLVLVSLTGLYASIINFEKLGGGASGGGGSGGGGSIQKTPQIQVYSRHPPENGKPNILNCYVTQFHPPHIEIQMLKNGKKIPKVEMSDMSFSKDWSFYILAHTEFTPTETDTYACRVKHASMAEPKTVYWDRDMGGGGSGGGGSGGGGSGGGGSGPHSLRYFVTAVSRPGLGEPRYMEVGYVDDTEFVRFDSDAENPRYEPRARWMEQEGPEYWERETQKAKGNEQSFRVDLRTLLGYYNQSKGGSHTIQVISGCEVGSDGRLLRGYQQYAYDGCDYIALNEDLKTWTAADMAALITKHKWEQAGEAERLRAYLEGTCVEWLRRYLKNGNATLLRTDSPKAHVTHHSRPEDKVTLRCWALGFYPADITLTWQLNGEELIQDMELVETRPAGDGTFQKWASVVVPLGKEQYYTCHVYHQGLPEPLTLRWEPPPSTVSNMATVAVLVVLGAAIVTGAVVAFVMKMRRRNTGGKGGDYALAPGSQTSDLSLPDCKVMVHDPHSLAMGVEGCTKCIKYLLFVFNFVFWLAGGVILGVALWLRHDPQTTSLLYLELGNKPAPNTFYVGIYILIAVGAVMMFVGFLGCYGAIQESQCLLGTFFTCLVILFACEVAAGIWGFVNKDQIAKDVKQFYDQALQQAVMDDDANNAKAVVKTFHETLNCCGSNALTTLTTTILRNSLCPSGGGGSAPTSSSTSSSTAEAQQQQQQQQQQQQHLEQLLMDLQELLSRMENYRNLKLPRMLTFKFYLPKQATELKDLQCLEDELGPLRHVLDLTQSKSFQLEDAENFISNIRVTVVKLKGSDNTFECQFDDESATVVDFLRRWIAFCQSIISTSPQGGGGSGGNILTPLLQQDCHQKIDELFSGKLYLIGIAAIVVAVIMIFEMILSMVLCCGIRNSSVY

SEQ ID NO: 136 - DNA, 2718 bp, Artificial Sequence
  sc-Trimer-CD81-IL-2
atggctcgctcggtgaccctggtctttctggtgcttgtctcactgaccggcctgtatgcttccattataaattttgaaaagttgggcggaggtgcctctggcggtgggggcagcggtggagggggcagtatccagaaaacccctcaaattcaagtatactcacgccacccaccggagaatgggaagccgaacatactgaactgctacgtaacacagttccacccgcctcacattgaaatccaaatgctgaagaacgggaaaaaaattcctaaagtagagatgtcagatatgtccttcagcaaggactggtctttctatatcctggctcacactgaattcacccccactgagactgatacatacgcctgcagagttaagcatgccagtatggccgagcccaagaccgtctactgggatcgagacatgggggggggaggctccggtggaggggggtctggagggggggggtctggtggaggcggaagtggcccacactcgctgaggtatttcgtcaccgccgtgtcccggcccggcctcggggagccccggtacatggaagtcggctacgtggacgacacggagttcgtgcgcttcgacagcgacgcggagaatccgagatatgagccgcgggcgcggtggatggagcaggaggggcccgagtattgggagcgggagacacagaaagccaagggcaatgagcagagtttccgagtggacctgaggaccctgctcggctactacaaccagagcaagggcggctctcacactattcaggtgatctctggctgtgaagtggggtccgacgggcgactcctccgcgggtaccagcagtacgcctacgacggctgcgattacatcgccctgaacgaagacctgaaaacgtggacggcggcggacatggcggcgctgatcaccaaacacaagtgggagcaggctggtgaagcagagagactcagggcctacctggagggcacgtgcgtggagtggctccgcagatacctgaagaacgggaacgcgacgctgctgcgcacagattccccaaaggcccatgtgacccatcacagcagacctgaagataaagtcaccctgaggtgctgggccctgggcttctaccctgctgacatcaccctgacctggcagttgaatggggaggagctgatccaggacatggagcttgtggagaccaggcctgcaggggatggaaccttccagaagtgggcatctgtggtggtgcctcttgggaaggagcagtattacacatgccatgtgtaccatcaggggctgcctgagcccctcaccctgagatgggagcctcctccatccactgtctccaacatggcgaccgttgctgttctggttgtccttggagctgcaatagtcactggagctgtggtggcttttgtgatgaagatgagaaggagaaacacaggtggaaaaggaggggactatgctctggctccaggctcccagacctctgatctgtctctcccagattgtaaagtgatggttcatgaccctcattctctagcgatgggggtggagggctgcaccaaatgcatcaaatacctgctcttcgtcttcaatttcgtcttctggctggctggaggcgtgatcctaggtgtagctctgtggttgcgtcatgatccacagaccaccagcctgctgtacctggaactgggaaacaaaccggcacccaacaccttctacgtgggcatctacattctcattgctgtgggagctgtgatgatgtttgtaggcttcctggggtgctatggggccatccaggagtcccagtgtctgctggggacgttcttcacctgccttgtgatcctgtttgcctgtgaggtggctgcaggcatctggggcttcgtaaacaaagaccagatcgccaaggatgtgaagcagttctatgaccaggcccttcagcaagctgtgatggatgatgatgccaacaatgccaaggctgtggtgaagactttccatgagacgctcaactgttgtggctccaacgcactgaccacactgactaccaccatactgaggaacagcctgtgtccctcaggaggaggaggaagcgcacccacttcaagctccacttcaagctctacagcggaagcacagcagcagcagcagcagcagcagcagcagcagcagcacctggagcagctgttgatggacctacaggagctcctgagcaggatggagaattacaggaacctgaaactccccaggatgctcaccttcaaattttacttgcccaagcaggccacagaattgaaagatcttcagtgcctagaagatgaacttggacctctgcggcatgttctggatttgactcaaagcaaaagctttcaattggaagatgctgagaatttcatcagcaatatcagagtaactgttgtaaaactaaagggctctgacaacacatttgagtgccaattcgatgatgagtcagcaactgtggtggactttctgaggagatggatagccttctgtcaaagcatcatctcaacaagccctcaaggaggaggaggaagcggcggcaacatactcacccccttactgcagcaagattgtcatcagaaaatcgatgagctcttctctgggaagctgtacctcattggaattgcagccattgtggtagctgtcattatgatctttgagatgattctgagcatggtgctgtgctgtggcatccggaacagctccgtgtactga

SEQ ID NO: 137 - protein, 550 aa, Artificial Sequence
  Aka-Luc
MEDAKNIKKGPAPFYPLEDGTAGEQLHKAMKRYALVPGAIAFTDAHIQVDVTYAEYFEMSVRLAEAMRRYGLNTNHRIVVCSENSSQFFMPVLGALFIGVAVAPANDIYNERELLNSMGISQPTVVFVSKKGLRKVLNVQKKLPIIRKIIIMDSKTDYQGFQSMYTFVTSHLPPSFNEYDFVPESFDRDKTIALIMNSSGSTGLPKGVALPHRTACVRFSHARDPIFGYQNIPDTAILSVVPFHHGFGMFTTLGYLICGFRVVLMYRFEEELFLRSLQDYKIQSALLVPTLFSCLAKSTLIDKYDLSSLREIASGGAPLSKEVGEAVAKRFRLPGIRQGYGLTETTNAVMITPEGDRKPGSVGKVVPFFEAKVVDLVTGKTLGVNQRGELCVRGPMIMSGYVNNPEATNALIDKDGWLHSGDIAYWDEDEHFFIVDRLKSLIKYKGYQVAPAELEGILLQHPYIFDAGVAGLPDDDAGELPAAVVVLEHGKTMTEKEIVDYVASQVTTAKKLRGGVVFVDEVPRGSTGKLDARKIREILTKAKKDGKIAV

SEQ ID NO: 138 - DNA, 1650 bp, Artificial Sequence
  Aka-Luc
atggaagatgccaaaaacattaagaagggcccagcgccgttctacccactcgaagacgggaccgccggcgagcagctgcacaaagccatgaagcgctacgccctggtgcccggcgccatcgcctttaccgacgcacatattcaggtggacgttacctacgccgagtacttcgagatgagcgttcggctggcagaagctatgaggcgctatgggctgaatacaaaccatcggatcgtggtgtgcagcgagaatagctcgcagttcttcatgcccgtgttgggtgccctgttcatcggtgtggctgtggccccagctaacgacatctacaacgagcgcgagctgctgaacagcatgggcatcagccagcccaccgtcgtattcgtgagcaagaaagggctgcgaaaggtcctcaacgtgcaaaagaagctaccgatcatacgaaagatcatcatcatggatagcaagaccgactaccagggcttccaaagcatgtacaccttcgtgacttcccatttgccacccagcttcaacgagtacgacttcgtgcccgagagcttcgaccgggacaaaaccatcgccctgatcatgaacagtagtggtagtacaggattacccaagggcgtagccctaccgcaccgcaccgcttgtgtccgattcagtcatgcccgcgaccccatcttcggctaccagaacatccccgacaccgctatcctcagcgtggtgccatttcaccacggcttcggcatgttcaccacgctgggctacttgatctgcggctttcgggtcgtgctcatgtaccgcttcgaggaggagctattcttgcgcagcttgcaagactataagattcaatctgccctgctggtgcccacactatttagctgcctcgctaagagcactctcatcgacaagtacgacctaagcagcttgcgcgagatcgccagcggcggggcgccgctcagcaaggaggtaggtgaggccgtggccaaacgcttccgcctaccaggcatccgccagggctatggcctgacagaaacaaccaacgccgtcatgatcacccccgagggggaccgtaagcctggctcagtaggcaaggtggtgcccttcttcgaggctaaggtggtagacttggtcaccggtaagacactgggtgtgaaccagcgcggtgagctgtgcgtccgtggccccatgatcatgagcggctacgttaacaaccccgaggctacgaacgctctcatcgacaaggacggctggctgcacagcggcgacatcgcctactgggacgaggacgagcacttcttcatcgtggaccggctgaagagcctgatcaaatacaagggctaccaggtagccccagccgaactggagggcatcctgctgcaacacccctacatcttcgacgccggagtcgccggcctgcccgacgacgatgccggcgagctgcccgccgcagtcgtcgtgttggaacacggtaaaaccatgaccgagaaagagatcgtggactatgtggccagccaggttacaaccgccaagaagctgcgcggtggtgttgtgtttgtggatgaagtccctagaggatcgaccggcaagttagacgcccgcaagatccgcgagattctcactaaggccaagaaggacggcaagatcgccgtg

SEQ ID NO: 139 - protein, 798 aa, Artificial Sequence
  CD63-Aka-Luc
MAVEGGMKCVKFLLYVLLLAFCACAVGLIAIGVAVQVVLKQAITHETTAGSLLPVVIIAVGAFLFLVAFVGCCGACKENYCLMITFAIFLSLIMLVEVAVAIAGYVFRDQVKSEFNKSFQQQMQNYLKDNKTATILDKLQKENNCCGASNYTDWENIPGMAKDRVPDSCCGGGGSMEDAKNIKKGPAPFYPLEDGTAGEQLHKAMKRYALVPGAIAFTDAHIQVDVTYAEYFEMSVRLAEAMRRYGLNTNHRIVVCSENSSQFFMPVLGALFIGVAVAPANDIYNERELLNSMGISQPTVVFVSKKGLRKVLNVQKKLPIIRKIIIMDSKTDYQGFQSMYTFVTSHLPPSFNEYDFVPESFDRDKTIALIMNSSGSTGLPKGVALPHRTACVRFSHARDPIFGYQNIPDTAILSVVPFHHGFGMFTTLGYLICGFRVVLMYRFEEELFLRSLQDYKIQSALLVPTLFSCLAKSTLIDKYDLSSLREIASGGAPLSKEVGEAVAKRFRLPGIRQGYGLTETTNAVMITPEGDRKPGSVGKVVPFFEAKVVDLVTGKTLGVNQRGELCVRGPMIMSGYVNNPEATNALIDKDGWLHSGDIAYWDEDEHFFIVDRLKSLIKYKGYQVAPAELEGILLQHPYIFDAGVAGLPDDDAGELPAAVVVLEHGKTMTEKEIVDYVASQVTTAKKLRGGVVFVDEVPRGSTGKLDARKIREILTKAKKDGKIAVGGGGSINITVGCGNDFKESTIHTQGCVETIAIWLRKNILLVAAAALGIAFVEVLGIIFSCCLVKSIRSGYEVM

SEQ ID NO: 140 - DNA, 2397 bp, Artificial Sequence
  CD63-Aka-Luc
atggcggtggaaggaggaatgaagtgtgtcaagtttttgctctacgttctcctgctggccttctgcgcctgtgcagtgggattgatcgccattggtgtagcggttcaggttgtcttgaagcaggccattacccatgagactactgctggctcgctgttgcctgtggtcatcattgcagtgggtgccttcctcttcctggtggcctttgtgggctgctgtggggcctgcaaggagaactactgtctcatgattacatttgccatcttcctgtctcttatcatgcttgtggaggtggctgtggccattgctggctatgtgtttagagaccaggtgaagtcagagtttaataaaagcttccagcagcagatgcagaattaccttaaagacaacaaaacagccactattttggacaaattgcagaaagaaaataactgctgtggagcttctaactacacagactgggaaaacatccccggcatggccaaggacagagtccccgattcttgctgcggtggtggtggttctatggaagatgccaaaaacattaagaagggcccagcgccgttctacccactcgaagacgggaccgccggcgagcagctgcacaaagccatgaagcgctacgccctggtgcccggcgccatcgcctttaccgacgcacatattcaggtggacgttacctacgccgagtacttcgagatgagcgttcggctggcagaagctatgaggcgctatgggctgaatacaaaccatcggatcgtggtgtgcagcgagaatagctcgcagttcttcatgcccgtgttgggtgccctgttcatcggtgtggctgtggccccagctaacgacatctacaacgagcgcgagctgctgaacagcatgggcatcagccagcccaccgtcgtattcgtgagcaagaaagggctgcgaaaggtcctcaacgtgcaaaagaagctaccgatcatacgaaagatcatcatcatggatagcaagaccgactaccagggcttccaaagcatgtacaccttcgtgacttcccatttgccacccagcttcaacgagtacgacttcgtgcccgagagcttcgaccgggacaaaaccatcgccctgatcatgaacagtagtggtagtacaggattacccaagggcgtagccctaccgcaccgcaccgcttgtgtccgattcagtcatgcccgcgaccccatcttcggctaccagaacatccccgacaccgctatcctcagcgtggtgccatttcaccacggcttcggcatgttcaccacgctgggctacttgatctgcggctttcgggtcgtgctcatgtaccgcttcgaggaggagctattcttgcgcagcttgcaagactataagattcaatctgccctgctggtgcccacactatttagctgcctcgctaagagcactctcatcgacaagtacgacctaagcagcttgcgcgagatcgccagcggcggggcgccgctcagcaaggaggtaggtgaggccgtggccaaacgcttccgcctaccaggcatccgccagggctatggcctgacagaaacaaccaacgccgtcatgatcacccccgagggggaccgtaagcctggctcagtaggcaaggtggtgcccttcttcgaggctaaggtggtagacttggtcaccggtaagacactgggtgtgaaccagcgcggtgagctgtgcgtccgtggccccatgatcatgagcggctacgttaacaaccccgaggctacgaacgctctcatcgacaaggacggctggctgcacagcggcgacatcgcctactgggacgaggacgagcacttcttcatcgtggaccggctgaagagcctgatcaaatacaagggctaccaggtagccccagccgaactggagggcatcctgctgcaacacccctacatcttcgacgccggagtcgccggcctgcccgacgacgatgccggcgagctgcccgccgcagtcgtcgtgttggaacacggtaaaaccatgaccgagaaagagatcgtggactatgtggccagccaggttacaaccgccaagaagctgcgcggtggtgttgtgtttgtggatgaagtccctagaggatcgaccggcaagttagacgcccgcaagatccgcgagattctcactaaggccaagaaggacggcaagatcgccgtgggtggtggtggttctatcaacataactgtgggctgtgggaatgatttcaaggaatccactatccatacccagggctgcgtggagactatagcaatatggctaaggaagaacatactgctggtggctgcagcggccctgggcattgcttttgtggaggtcttgggaattatcttctcctgctgtctggtgaagagtattcgaagtggctatgaagtaatgtag

SEQ ID NO: 141 - protein, 9 aa, Artificial Sequence
  SAR-CoV2 peptide
KLWAQCVQL

SEQ ID NO: 142 - DNA, 27 bp, Artificial Sequence
  SARS-CoV2 DNA
aaactgtgggcccagtgtgtgcagctg

SEQ ID NO: 143 - protein, 341 aa, Artificial Sequence
  HLA-A0201
GSHSMRYFFTSVSRPGRGEPRFIAVGYVDDTQFVRFDSDAASQRMEPRAPWIEQEGPEYWDGETRKVKAHSQTHRVDLGTLRGYYNQSEAGSHTVQRMYGCDVGSDWRFLRGYHQYAYDGKDYIALKEDLRSWTAADMAAQTTKHKWEAAHVAEQLRAYLEGTCVEWLRRYLENGKETLQRTDAPKTHMTHHAVSDHEATLRCWALSFYPAEITLTWQRDGEDQTQDTELVETRPAGDGTFQKWAAVVVPSGQEQRYTCHVQHEGLPKPLTLRWEPSSQPTIPIVGIIAGLVLFGAVITGAVVAAVMWRRKSSDRKGGSYSQAASSDSAQGSDVSLTACKV

SEQ ID NO: 144 - DNA, 1023 bp, Artificial Sequence
  HLA-A0201
ggctctcactccatgaggtatttcttcacatccgtgtcccggcccggccgcggggagccccgcttcatcgcagtgggctacgtggacgacacgcagttcgtgcggttcgacagcgacgccgcgagccagaggatggagccgcgggcgccgtggatagagcaggagggtccggagtattgggacggggagacacggaaagtgaaggcccactcacagactcaccgagtggacctggggaccctgcgcggctactacaaccagagcgaggccggttctcacaccgtccagaggatgtatggctgcgacgtggggtcggactggcgcttcctccgcgggtaccaccagtacgcctacgacggcaaggattacatcgccctgaaagaggacctgcgctcttggaccgcggcggacatggcagctcagaccaccaagcacaagtgggaggcggcccatgtggcggagcagttgagagcctacctggagggcacgtgcgtggagtggctccgcagatacctggagaacgggaaggagacgctgcagcgcacggacgcccccaaaacgcatatgactcaccacgctgtctctgaccatgaagccaccctgaggtgctgggccctgagcttctaccctgcggagatcacactgacctggcagcgggatggggaggaccagacccaggacacggagctcgtggagaccaggcctgcaggggatggaaccttccagaagtgggcggctgtggtggtgccttctggacaggagcagagatacacctgccatgtgcagcatgagggtttgcccaagcccctcaccctgagatgggagccgtcttcccagcccaccatccccatcgtgggcatcattgctggcctggttctctttggagctgtgatcactggagctgtggtcgctgctgtgatgtggaggaggaagagctcagatagaaaaggagggagctactctcaggctgcaagcagtgacagtgcccagggctctgatgtgtctctcacagcttgtaaagtg

SEQ ID NO: 145 - protein, 460 aa, Artificial Sequence
  hsMHC-I
IQRTPKIQVYSRHPAENGKSNFLNCYVSGFHPSDIEVDLLKNGERIEKVEHSDLSFSKDWSFYLLYYTEFTPTEKDEYACRVNHVTLSQPKIVKWDRDMGGGGSGGGGSGGGGSGGGGSGSHSMRYFFTSVSRPGRGEPRFIAVGYVDDTQFVRFDSDAASQRMEPRAPWIEQEGPEYWDGETRKVKAHSQTHRVDLGTLRGYYNQSEAGSHTVQRMYGCDVGSDWRFLRGYHQYAYDGKDYIALKEDLRSWTAADMAAQTTKHKWEAAHVAEQLRAYLEGTCVEWLRRYLENGKETLQRTDAPKTHMTHHAVSDHEATLRCWALSFYPAEITLTWQRDGEDQTQDTELVETRPAGDGTFQKWAAVVVPSGQEQRYTCHVQHEGLPKPLTLRWEPSSQPTIPIVGIIAGLVLFGAVITGAVVAAVMWRRKSSDRKGGSYSQAASSDSAQGSDVSLTACKV

SEQ ID NO: 146 - DNA, 1380 bp, Artificial Sequence
  hsMHC-I
atccagcgtactccaaagattcaggtttactcacgtcatccagcagagaatggaaagtcaaatttcctgaattgctatgtgtctgggtttcatccatccgacattgaagttgacttactgaagaatggagagagaattgaaaaagtggagcattcagacttgtctttcagcaaggactggtctttctatctcttgtactacactgaattcacccccactgaaaaagatgagtatgcctgccgtgtgaaccatgtgactttgtcacagcccaagatagttaagtgggatcgagacatgggaggcggcgggtctggcggcggcggcagtggcggtggcggtagcggcggaggtggatctggctctcactccatgaggtatttcttcacatccgtgtcccggcccggccgcggggagccccgcttcatcgcagtgggctacgtggacgacacgcagttcgtgcggttcgacagcgacgccgcgagccagaggatggagccgcgggcgccgtggatagagcaggagggtccggagtattgggacggggagacacggaaagtgaaggcccactcacagactcaccgagtggacctggggaccctgcgcggctactacaaccagagcgaggccggttctcacaccgtccagaggatgtatggctgcgacgtggggtcggactggcgcttcctccgcgggtaccaccagtacgcctacgacggcaaggattacatcgccctgaaagaggacctgcgctcttggaccgcggcggacatggcagctcagaccaccaagcacaagtgggaggcggcccatgtggcggagcagttgagagcctacctggagggcacgtgcgtggagtggctccgcagatacctggagaacgggaaggagacgctgcagcgcacggacgcccccaaaacgcatatgactcaccacgctgtctctgaccatgaagccaccctgaggtgctgggccctgagcttctaccctgcggagatcacactgacctggcagcgggatggggaggaccagacccaggacacggagctcgtggagaccaggcctgcaggggatggaaccttccagaagtgggcggctgtggtggtgccttctggacaggagcagagatacacctgccatgtgcagcatgagggtttgcccaagcccctcaccctgagatgggagccgtcttcccagcccaccatccccatcgtgggcatcattgctggcctggttctctttggagctgtgatcactggagctgtggtcgctgctgtgatgtggaggaggaagagctcagatagaaaaggagggagctactctcaggctgcaagcagtgacagtgcccagggctctgatgtgtctctcacagcttgtaaagtg

SEQ ID NO: 147 - protein, 504 aa, Artificial Sequence
  SARS-CoV2sc-Trimer
MSRSVALAVLALLSLSGLEAKLWAQCVQLGGGASGGGGSGGGGSIQRTPKIQVYSRHPAENGKSNFLNCYVSGFHPSDIEVDLLKNGERIEKVEHSDLSFSKDWSFYLLYYTEFTPTEKDEYACRVNHVTLSQPKIVKWDRDMGGGGSGGGGSGGGGSGGGGSGSHSMRYFFTSVSRPGRGEPRFIAVGYVDDTQFVRFDSDAASQRMEPRAPWIEQEGPEYWDGETRKVKAHSQTHRVDLGTLRGYYNQSEAGSHTVQRMYGCDVGSDWRFLRGYHQYAYDGKDYIALKEDLRSWTAADMAAQTTKHKWEAAHVAEQLRAYLEGTCVEWLRRYLENGKETLQRTDAPKTHMTHHAVSDHEATLRCWALSFYPAEITLTWQRDGEDQTQDTELVETRPAGDGTFQKWAAVVVPSGQEQRYTCHVQHEGLPKPLTLRWEPSSQPTIPIVGIIAGLVLFGAVITGAVVAAVMWRRKSSDRKGGSYSQAASSDSAQGSDVSLTACKV

SEQ ID NO: 148 - DNA, 1512 bp, Artificial Sequence
  SARS-CoV2sc-Trimer
atgtctcgctccgtggccttagctgtgctcgcgctactctctctttctggcctggaggctaaactgtgggcccagtgtgtgcagctgggcggaggggcatcaggcggcggtgggtcaggtggaggtgggagtatccagcgtactccaaagattcaggtttactcacgtcatccagcagagaatggaaagtcaaatttcctgaattgctatgtgtctgggtttcatccatccgacattgaagttgacttactgaagaatggagagagaattgaaaaagtggagcattcagacttgtctttcagcaaggactggtctttctatctcttgtactacactgaattcacccccactgaaaaagatgagtatgcctgccgtgtgaaccatgtgactttgtcacagcccaagatagttaagtgggatcgagacatgggaggcggcgggtctggcggcggcggcagtggcggtggcggtagcggcggaggtggatctggctctcactccatgaggtatttcttcacatccgtgtcccggcccggccgcggggagccccgcttcatcgcagtgggctacgtggacgacacgcagttcgtgcggttcgacagcgacgccgcgagccagaggatggagccgcgggcgccgtggatagagcaggagggtccggagtattgggacggggagacacggaaagtgaaggcccactcacagactcaccgagtggacctggggaccctgcgcggctactacaaccagagcgaggccggttctcacaccgtccagaggatgtatggctgcgacgtggggtcggactggcgcttcctccgcgggtaccaccagtacgcctacgacggcaaggattacatcgccctgaaagaggacctgcgctcttggaccgcggcggacatggcagctcagaccaccaagcacaagtgggaggcggcccatgtggcggagcagttgagagcctacctggagggcacgtgcgtggagtggctccgcagatacctggagaacgggaaggagacgctgcagcgcacggacgcccccaaaacgcatatgactcaccacgctgtctctgaccatgaagccaccctgaggtgctgggccctgagcttctaccctgcggagatcacactgacctggcagcgggatggggaggaccagacccaggacacggagctcgtggagaccaggcctgcaggggatggaaccttccagaagtgggcggctgtggtggtgccttctggacaggagcagagatacacctgccatgtgcagcatgagggtttgcccaagcccctcaccctgagatgggagccgtcttcccagcccaccatccccatcgtgggcatcattgctggcctggttctctttggagctgtgatcactggagctgtggtcgctgctgtgatgtggaggaggaagagctcagatagaaaaggagggagctactctcaggctgcaagcagtgacagtgcccagggctctgatgtgtctctcacagcttgtaaagtg

SEQ ID NO: 149 - protein, 740 aa, Artificial Sequence
  SARS-CoV2sc-Trimer-CD81
MSRSVALAVLALLSLSGLEAKLWAQCVQLGGGASGGGGSGGGGSIQRTPKIQVYSRHPAENGKSNFLNCYVSGFHPSDIEVDLLKNGERIEKVEHSDLSFSKDWSFYLLYYTEFTPTEKDEYACRVNHVTLSQPKIVKWDRDMGGGGSGGGGSGGGGSGGGGSGSHSMRYFFTSVSRPGRGEPRFIAVGYVDDTQFVRFDSDAASQRMEPRAPWIEQEGPEYWDGETRKVKAHSQTHRVDLGTLRGYYNQSEAGSHTVQRMYGCDVGSDWRFLRGYHQYAYDGKDYIALKEDLRSWTAADMAAQTTKHKWEAAHVAEQLRAYLEGTCVEWLRRYLENGKETLQRTDAPKTHMTHHAVSDHEATLRCWALSFYPAEITLTWQRDGEDQTQDTELVETRPAGDGTFQKWAAVVVPSGQEQRYTCHVQHEGLPKPLTLRWEPSSQPTIPIVGIIAGLVLFGAVITGAVVAAVMWRRKSSDRKGGSYSQAASSDSAQGSDVSLTACKVMGVEGCTKCIKYLLFVFNFVFWLAGGVILGVALWLRHDPQTTNLLYLELGDKPAPNTFYVGIYILIAVGAVMMFVGFLGCYGAIQESQCLLGTFFTCLVILFACEVAAGIWGFVNKDQIAKDVKQFYDQALQQAVVDDDANNAKAVVKTFHETLDCCGSSTLTALTTSVLKNNLCPSGSNIISNLFKEDCHQKIDDLFSGKLYLIGIAAIVVAVIMIFEMILSMVLCCGIRNSSVY

SEQ ID NO: 150 - DNA, 2223 bp, Artificial Sequence
  SARS-CoV2sc-Trimer-CD81
atgtctcgctccgtggccttagctgtgctcgcgctactctctctttctggcctggaggctaaactgtgggcccagtgtgtgcagctgggcggaggggcatcaggcggcggtgggtcaggtggaggtgggagtatccagcgtactccaaagattcaggtttactcacgtcatccagcagagaatggaaagtcaaatttcctgaattgctatgtgtctgggtttcatccatccgacattgaagttgacttactgaagaatggagagagaattgaaaaagtggagcattcagacttgtctttcagcaaggactggtctttctatctcttgtactacactgaattcacccccactgaaaaagatgagtatgcctgccgtgtgaaccatgtgactttgtcacagcccaagatagttaagtgggatcgagacatgggaggcggcgggtctggcggcggcggcagtggcggtggcggtagcggcggaggtggatctggctctcactccatgaggtatttcttcacatccgtgtcccggcccggccgcggggagccccgcttcatcgcagtgggctacgtggacgacacgcagttcgtgcggttcgacagcgacgccgcgagccagaggatggagccgcgggcgccgtggatagagcaggagggtccggagtattgggacggggagacacggaaagtgaaggcccactcacagactcaccgagtggacctggggaccctgcgcggctactacaaccagagcgaggccggttctcacaccgtccagaggatgtatggctgcgacgtggggtcggactggcgcttcctccgcgggtaccaccagtacgcctacgacggcaaggattacatcgccctgaaagaggacctgcgctcttggaccgcggcggacatggcagctcagaccaccaagcacaagtgggaggcggcccatgtggcggagcagttgagagcctacctggagggcacgtgcgtggagtggctccgcagatacctggagaacgggaaggagacgctgcagcgcacggacgcccccaaaacgcatatgactcaccacgctgtctctgaccatgaagccaccctgaggtgctgggccctgagcttctaccctgcggagatcacactgacctggcagcgggatggggaggaccagacccaggacacggagctcgtggagaccaggcctgcaggggatggaaccttccagaagtgggcggctgtggtggtgccttctggacaggagcagagatacacctgccatgtgcagcatgagggtttgcccaagcccctcaccctgagatgggagccgtcttcccagcccaccatccccatcgtgggcatcattgctggcctggttctctttggagctgtgatcactggagctgtggtcgctgctgtgatgtggaggaggaagagctcagatagaaaaggagggagctactctcaggctgcaagcagtgacagtgcccagggctctgatgtgtctctcacagcttgtaaagtgatgggagtggagggctgcaccaagtgcatcaagtacctgctcttcgtcttcaatttcgtcttctggctggctggaggcgtgatcctgggtgtggccctgtggctccgccatgacccgcagaccaccaacctcctgtatctggagctgggagacaagcccgcgcccaacaccttctatgtaggcatctacatcctcatcgctgtgggcgctgtcatgatgttcgttggcttcctgggctgctacggggccatccaggaatcccagtgcctgctggggacgttcttcacctgcctggtcatcctgtttgcctgtgaggtggccgccggcatctggggctttgtcaacaaggaccagatcgccaaggatgtgaagcagttctatgaccaggccctacagcaggccgtggtggatgatgacgccaacaacgccaaggctgtggtgaagaccttccacgagacgcttgactgctgtggctccagcacactgactgctttgaccacctcagtgctcaagaacaatttgtgtccctcgggcagcaacatcatcagcaacctcttcaaggaggactgccaccagaagatcgatgacctcttctccgggaagctgtacctcatcggcattgctgccatcgtggtcgctgtgatcatgatcttcgagatgatcctgagcatggtgctgtgctgtggcatccggaacagctccgtgtactga